European Patent Application EP 4 227 411 A1, published August 16, 2023. Title: An engineered guide RNA for the optimized CRISPR/Cas12f1 system and use thereof. Applicant: Genkore. The sequence listing filed with the application follows.

SEQUENCE LISTING (441 sequences)

SEQ ID NO: 1 - RNA, 140 nt, Artificial Sequence
  mature form of Cas12f1 tracrRNA
cuucacugauaaaguggagaaccgcuucaccaaaagcugucccuuaggggauuagaacuugagugaaggugggcugcuugcaucagccuaaugucgagaagugcuuucuucggaaaguaacccucgaaacaaauucauuu

SEQ ID NO: 2 - RNA, 161 nt, Artificial Sequence
  wild-type of Cas12f1 tracrRNA
cuucacugauaaaguggagaaccgcuucaccaaaagcugucccuuaggggauuagaacuugagugaaggugggcugcuugcaucagccuaaugucgagaagugcuuucuucggaaaguaacccucgaaacaaauucauuuuuccucuccaauucugcacaa

SEQ ID NO: 3 - RNA, 17 nt, Artificial Sequence
  mature form of Cas12f1 crRNA repeat
gaaugaaggaaugcaac

SEQ ID NO: 4 - RNA, 37 nt, Artificial Sequence
  wild-type of Cas12f1 crRNA repeat
guugcagaacccgaauagacgaaugaaggaaugcaac

SEQ ID NO: 5 - RNA, 37 nt, Artificial Sequence
  mature form of Cas12f1 crRNA
gaaugaaggaaugcaacnnnnnnnnnnnnnnnnnnnn

SEQ ID NO: 6 - RNA, 57 nt, Artificial Sequence
  wild-type of Cas12f1 crRNA
guugcagaacccgaauagacgaaugaaggaaugcaacnnnnnnnnnnnnnnnnnnnn

SEQ ID NO: 7 - RNA, 161 nt, Artificial Sequence
  mature form of Cas12f1 tracrRNA + GAAA + mature form of Cas12f1 crRNA repeat
cuucacugauaaaguggagaaccgcuucaccaaaagcugucccuuaggggauuagaacuugagugaaggugggcugcuugcaucagccuaaugucgagaagugcuuucuucggaaaguaacccucgaaacaaauucauuugaaagaaugaaggaaugcaac

SEQ ID NO: 8 - RNA, 181 nt, Artificial Sequence
  mature form of Cas12f1 tracrRNA + GAAA + mature form of Cas12f1 crRNA
cuucacugauaaaguggagaaccgcuucaccaaaagcugucccuuaggggauuagaacuugagugaaggugggcugcuugcaucagccuaaugucgagaagugcuuucuucggaaaguaacccucgaaacaaauucauuugaaagaaugaaggaaugcaacnnnnnnnnnnnnnnnnnnnn

SEQ ID NO: 9 - RNA, 21 nt, Artificial Sequence
  1st region of Cas12f1 guide RNA
cuucacugauaaaguggagaa

SEQ ID NO: 10 - RNA, 50 nt, Artificial Sequence
  2nd region of Cas12f1 guide RNA
ccgcuucaccaaaagcugucccuuaggggauuagaacuugagugaaggug

SEQ ID NO: 11 - RNA, 56 nt, Artificial Sequence
  3rd region of Cas12f1 guide RNA
ggcugcuugcaucagccuaaugucgagaagugcuuucuucggaaaguaacccucga

SEQ ID NO: 12 - RNA, 13 nt, Artificial Sequence
  4th region of Cas12f1 guide RNA (Mature form)
aacaaauucauuu

SEQ ID NO: 13 - RNA, 34 nt, Artificial Sequence
  4th region of Cas12f1 guide RNA (Wild-type)
aacaaauucauuuuuccucuccaauucugcacaa

SEQ ID NO: 14 - RNA, 10 nt, Artificial Sequence
  5th region of Cas12f1 guide RNA (Mature form)
gaaugaagga

SEQ ID NO: 15 - RNA, 30 nt, Artificial Sequence
  5th region of Cas12f1 guide RNA (Wild-type)
guugcagaacccgaauagacgaaugaagga

SEQ ID NO: 16 - RNA, 10 nt, Artificial Sequence
  first region, 11nt deletion
aaguggagaa

SEQ ID NO: 17 - RNA, 11 nt, Artificial Sequence
  first region, 10nt deletion
aaaguggagaa

SEQ ID NO: 18 - RNA, 12 nt, Artificial Sequence
  first region, 9nt deletion
uaaaguggagaa

SEQ ID NO: 19 - RNA, 13 nt, Artificial Sequence
  first region, 8nt deletion
auaaaguggagaa

SEQ ID NO: 20 - RNA, 14 nt, Artificial Sequence
  first region, 7nt deletion
gauaaaguggagaa

SEQ ID NO: 21 - RNA, 15 nt, Artificial Sequence
  first region, 6nt deletion
ugauaaaguggagaa

SEQ ID NO: 22 - RNA, 16 nt, Artificial Sequence
  first region, 5nt deletion
cugauaaaguggagaa

SEQ ID NO: 23 - RNA, 17 nt, Artificial Sequence
  first region, 4nt deletion
acugauaaaguggagaa

SEQ ID NO: 24 - RNA, 18 nt, Artificial Sequence
  first region, 3nt deletion
cacugauaaaguggagaa

SEQ ID NO: 25 - RNA, 19 nt, Artificial Sequence
  first region, 2nt deletion
ucacugauaaaguggagaa

SEQ ID NO: 26 - RNA, 20 nt, Artificial Sequence
  first region, 1nt deletion
uucacugauaaaguggagaa

SEQ ID NO: 27 - RNA, 10 nt, Artificial Sequence
  deleted part of the first region, 10nt
aaaguggaga

SEQ ID NO: 28 - RNA, 11 nt, Artificial Sequence
  deleted part of the first region, 11nt
uaaaguggaga

SEQ ID NO: 29 - RNA, 12 nt, Artificial Sequence
  deleted part of the first region, 12nt
auaaaguggaga

SEQ ID NO: 30 - RNA, 13 nt, Artificial Sequence
  deleted part of the first region, 13nt
gauaaaguggaga

SEQ ID NO: 31 - RNA, 14 nt, Artificial Sequence
  deleted part of the first region, 14nt
ugauaaaguggaga

SEQ ID NO: 32 - RNA, 15 nt, Artificial Sequence
  deleted part of the first region, 15nt
cugauaaaguggaga

SEQ ID NO: 33 - RNA, 16 nt, Artificial Sequence
  deleted part of the first region, 16nt
acugauaaaguggaga

SEQ ID NO: 34 - RNA, 17 nt, Artificial Sequence
  deleted part of the first region, 17nt
cacugauaaaguggaga

SEQ ID NO: 35 - RNA, 18 nt, Artificial Sequence
  deleted part of the first region, 18nt
ucacugauaaaguggaga

SEQ ID NO: 36 - RNA, 19 nt, Artificial Sequence
  deleted part of the first region, 19nt
uucacugauaaaguggaga

SEQ ID NO: 37 - RNA, 20 nt, Artificial Sequence
  deleted part of the first region, 20nt
cuucacugauaaaguggaga

SEQ ID NO: 38 - RNA, 28 nt, Artificial Sequence
  second region, 11bp deletion
ccgcuucaccauuagugagugaaggugg

SEQ ID NO: 39 - RNA, 30 nt, Artificial Sequence
  second region, 10bp deletion
ccgcuucaccaauuaguugagugaaggugg

SEQ ID NO: 40 - RNA, 32 nt, Artificial Sequence
  second region, 9bp deletion
ccgcuucaccaaauuagcuugagugaaggugg

SEQ ID NO: 41 - RNA, 34 nt, Artificial Sequence
  second region, 8bp deletion
ccgcuucaccaaaauuagacuugagugaaggugg

SEQ ID NO: 42 - RNA, 36 nt, Artificial Sequence
  second region, 7bp deletion
ccgcuucaccaaaaguuagaacuugagugaaggugg

SEQ ID NO: 43 - RNA, 38 nt, Artificial Sequence
  second region, 6bp deletion
ccgcuucaccaaaagcuuaggaacuugagugaaggugg

SEQ ID NO: 44 - RNA, 40 nt, Artificial Sequence
  second region, 5bp deletion
ccgcuucaccaaaagcuuuagagaacuugagugaaggugg

SEQ ID NO: 45 - RNA, 43 nt, Artificial Sequence
  second region, 4bp deletion
ccgcuucaccaaaagcuguuaguuagaacuugagugaaggugg

SEQ ID NO: 46 - RNA, 42 nt, Artificial Sequence
  second region, 4bp+1nt deletion
ccgcuucaccaaaagcuguuaguagaacuugagugaaggugg

SEQ ID NO: 47 - RNA, 45 nt, Artificial Sequence
  second region, 3bp deletion
ccgcuucaccaaaagcuguuuagauuagaacuugagugaaggugg

SEQ ID NO: 48 - RNA, 47 nt, Artificial Sequence
  second region, 2bp deletion
ccgcuucaccaaaagcugucuuaggauuagaacuugagugaaggugg

SEQ ID NO: 49 - RNA, 49 nt, Artificial Sequence
  second region, 1bp deletion
ccgcuucaccaaaagcuguccuuagggauuagaacuugagugaaggugg

SEQ ID NO: 50 - RNA, 11 nt, Artificial Sequence
  second region, 5' remains
ccgcuucacca

SEQ ID NO: 51 - RNA, 13 nt, Artificial Sequence
  second region, 3' remains
ugagugaaggugg

SEQ ID NO: 52 - RNA, 10 nt, Artificial Sequence
  upper-deleted part of the second region, 10nt
aaagcugucc

SEQ ID NO: 53 - RNA, 11 nt, Artificial Sequence
  upper-deleted part of the second region, 11nt
aaagcuguccc

SEQ ID NO: 54 - RNA, 10 nt, Artificial Sequence
  lower-deleted part of the second region, 10nt
gauuagaacu

SEQ ID NO: 55 - RNA, 11 nt, Artificial Sequence
  lower-deleted part of the second region, 11nt
ggauuagaacu

SEQ ID NO: 56 - RNA, 12 nt, Artificial Sequence
  lower-deleted part of the second region, 12nt
gggauuagaacu

SEQ ID NO: 57 - RNA, 10 nt, Artificial Sequence
  intermediate sequence of the second region, 10nt
aaauuagacu

SEQ ID NO: 58 - RNA, 12 nt, Artificial Sequence
  intermediate sequence of the second region, 11nt
aaaguuagaacu

SEQ ID NO: 59 - RNA, 14 nt, Artificial Sequence
  intermediate sequence of the second region, 12nt
aaagcuuaggaacu

SEQ ID NO: 60 - RNA, 16 nt, Artificial Sequence
  intermediate sequence of the second region, 13nt
aaagcuuuagagaacu

SEQ ID NO: 61 - RNA, 18 nt, Artificial Sequence
  intermediate sequence of the second region, 14nt
aaagcuguuaguagaacu

SEQ ID NO: 62 - RNA, 19 nt, Artificial Sequence
  intermediate sequence of the second region, 15nt
aaagcuguuaguuagaacu

SEQ ID NO: 63 - RNA, 21 nt, Artificial Sequence
  intermediate sequence of the second region, 16nt
aaagcuguuuagauuagaacu

SEQ ID NO: 64 - RNA, 23 nt, Artificial Sequence
  intermediate sequence of the second region, 17nt
aaagcugucuuaggauuagaacu

SEQ ID NO: 65 - RNA, 25 nt, Artificial Sequence
  intermediate sequence of the second region, 18nt
aaagcuguccuuagggauuagaacu

SEQ ID NO: 66 - RNA, 10 nt, Artificial Sequence
  fourth region of the tracrRNA(mature form), delete 3nt
aacaaauuca

SEQ ID NO: 67 - RNA, 11 nt, Artificial Sequence
  fourth region of the tracrRNA(mature form), delete 4nt
aacaaauucau

SEQ ID NO: 68 - RNA, 12 nt, Artificial Sequence
  fourth region of the tracrRNA(mature form), delete 5nt
aacaaauucauu

SEQ ID NO: 69 - RNA, 13 nt, Artificial Sequence
  fourth region of the tracrRNA(wild-type), 21nt deletion
aacaaauucauuu

SEQ ID NO: 70 - RNA, 14 nt, Artificial Sequence
  fourth region of the tracrRNA(wild-type), 20nt deletion
aacaaauucauuuu

SEQ ID NO: 71 - RNA, 15 nt, Artificial Sequence
  fourth region of the tracrRNA(wild-type), 19nt deletion
aacaaauucauuuuu

SEQ ID NO: 72 - RNA, 16 nt, Artificial Sequence
  fourth region of the tracrRNA(wild-type), 18nt deletion
aacaaauucauuuuuc

SEQ ID NO: 73 - RNA, 17 nt, Artificial Sequence
  fourth region of the tracrRNA(wild-type), 17nt deletion
aacaaauucauuuuucc

SEQ ID NO: 74 - RNA, 18 nt, Artificial Sequence
  fourth region of the tracrRNA(wild-type), 16nt deletion
aacaaauucauuuuuccu

SEQ ID NO: 75 - RNA, 19 nt, Artificial Sequence
  fourth region of the tracrRNA(wild-type), 15nt deletion
aacaaauucauuuuuccuc

SEQ ID NO: 76 - RNA, 20 nt, Artificial Sequence
  fourth region of the tracrRNA(wild-type), 14nt deletion
aacaaauucauuuuuccucu

SEQ ID NO: 77 - RNA, 21 nt, Artificial Sequence
  fourth region of the tracrRNA(wild-type), 13nt deletion
aacaaauucauuuuuccucuc

SEQ ID NO: 78 - RNA, 22 nt, Artificial Sequence
  fourth region of the tracrRNA(wild-type), 12nt deletion
aacaaauucauuuuuccucucc

SEQ ID NO: 79 - RNA, 23 nt, Artificial Sequence
  fourth region of the tracrRNA(wild-type), 11nt deletion
aacaaauucauuuuuccucucca

SEQ ID NO: 80 - RNA, 24 nt, Artificial Sequence
  fourth region of the tracrRNA(wild-type), 10nt deletion
aacaaauucauuuuuccucuccaa

SEQ ID NO: 81 - RNA, 25 nt, Artificial Sequence
  fourth region of the tracrRNA(wild-type), 9nt deletion
aacaaauucauuuuuccucuccaau

SEQ ID NO: 82 - RNA, 26 nt, Artificial Sequence
  fourth region of the tracrRNA(wild-type), 8nt deletion
aacaaauucauuuuuccucuccaauu

SEQ ID NO: 83 - RNA, 27 nt, Artificial Sequence
  fourth region of the tracrRNA(wild-type), 7nt deletion
aacaaauucauuuuuccucuccaauuc

SEQ ID NO: 84 - RNA, 28 nt, Artificial Sequence
  fourth region of the tracrRNA(wild-type), 6nt deletion
aacaaauucauuuuuccucuccaauucu

SEQ ID NO: 85 - RNA, 29 nt, Artificial Sequence
  fourth region of the tracrRNA(wild-type), 5nt deletion
aacaaauucauuuuuccucuccaauucug

SEQ ID NO: 86 - RNA, 30 nt, Artificial Sequence
  fourth region of the tracrRNA(wild-type), 4nt deletion
aacaaauucauuuuuccucuccaauucugc

SEQ ID NO: 87 - RNA, 31 nt, Artificial Sequence
  fourth region of the tracrRNA(wild-type), 3nt deletion
aacaaauucauuuuuccucuccaauucugca

SEQ ID NO: 88 - RNA, 32 nt, Artificial Sequence
  fourth region of the tracrRNA(wild-type), 2nt deletion
aacaaauucauuuuuccucuccaauucugcac

SEQ ID NO: 89 - RNA, 33 nt, Artificial Sequence
  fourth region of the tracrRNA(wild-type), 1nt deletion
aacaaauucauuuuuccucuccaauucugcaca

SEQ ID NO: 90 - RNA, 10 nt, Artificial Sequence
  fifth region of the crRNA(wild-type), 20nt deletion
gaaugaagga

SEQ ID NO: 91 - RNA, 11 nt, Artificial Sequence
  fifth region of the crRNA(wild-type), 19nt deletion
cgaaugaagga

SEQ ID NO: 92 - RNA, 12 nt, Artificial Sequence
  fifth region of the crRNA(wild-type), 18nt deletion
acgaaugaagga

SEQ ID NO: 93 - RNA, 13 nt, Artificial Sequence
  fifth region of the crRNA(wild-type), 17nt deletion
gacgaaugaagga

SEQ ID NO: 94 - RNA, 14 nt, Artificial Sequence
  fifth region of the crRNA(wild-type), 16nt deletion
agacgaaugaagga

SEQ ID NO: 95 - RNA, 15 nt, Artificial Sequence
  fifth region of the crRNA(wild-type), 15nt deletion
uagacgaaugaagga

SEQ ID NO: 96 - RNA, 16 nt, Artificial Sequence
  fifth region of the crRNA(wild-type), 14nt deletion
auagacgaaugaagga

SEQ ID NO: 97 - RNA, 17 nt, Artificial Sequence
  fifth region of the crRNA(wild-type), 13nt deletion
aauagacgaaugaagga

SEQ ID NO: 98 - RNA, 18 nt, Artificial Sequence
  fifth region of the crRNA(wild-type), 12nt deletion
gaauagacgaaugaagga

SEQ ID NO: 99 - RNA, 19 nt, Artificial Sequence
  fifth region of the crRNA(wild-type), 11nt deletion
cgaauagacgaaugaagga

SEQ ID NO: 100 - RNA, 20 nt, Artificial Sequence
  fifth region of the crRNA(wild-type), 10nt deletion
ccgaauagacgaaugaagga

SEQ ID NO: 101 - RNA, 21 nt, Artificial Sequence
  fifth region of the crRNA(wild-type), 9nt deletion
cccgaauagacgaaugaagga

SEQ ID NO: 102 - RNA, 22 nt, Artificial Sequence
  fifth region of the crRNA(wild-type), 8nt deletion
acccgaauagacgaaugaagga

SEQ ID NO: 103 - RNA, 23 nt, Artificial Sequence
  fifth region of the crRNA(wild-type), 7nt deletion
aacccgaauagacgaaugaagga

SEQ ID NO: 104 - RNA, 24 nt, Artificial Sequence
  fifth region of the crRNA(wild-type), 6nt deletion
gaacccgaauagacgaaugaagga

SEQ ID NO: 105 - RNA, 25 nt, Artificial Sequence
  fifth region of the crRNA(wild-type), 5nt deletion
agaacccgaauagacgaaugaagga

SEQ ID NO: 106 - RNA, 26 nt, Artificial Sequence
  fifth region of the crRNA(wild-type), 4nt deletion
cagaacccgaauagacgaaugaagga

SEQ ID NO: 107 - RNA, 27 nt, Artificial Sequence
  fifth region of the crRNA(wild-type), 3nt deletion
gcagaacccgaauagacgaaugaagga

SEQ ID NO: 108 - RNA, 28 nt, Artificial Sequence
  fifth region of the crRNA(wild-type), 2nt deletion
ugcagaacccgaauagacgaaugaagga

SEQ ID NO: 109 - RNA, 29 nt, Artificial Sequence
  fifth region of the crRNA(wild-type), 1nt deletion
uugcagaacccgaauagacgaaugaagga

SEQ ID NO: 110 - RNA, 13 nt, Artificial Sequence
  fourth region + Linker + fifth region, 7bp deletion (mature form)
aacaaagaaagga

SEQ ID NO: 111 - RNA, 15 nt, Artificial Sequence
  fourth region + Linker + fifth region, 6bp deletion (mature form)
aacaaaugaaaagga

SEQ ID NO: 112 - RNA, 17 nt, Artificial Sequence
  fourth region + Linker + fifth region, 5bp deletion (mature form)
aacaaauugaaaaagga

SEQ ID NO: 113 - RNA, 19 nt, Artificial Sequence
  fourth region + Linker + fifth region, 4bp deletion (mature form)
aacaaauucgaaagaagga

SEQ ID NO: 114 - RNA, 21 nt, Artificial Sequence
  fourth region + Linker + fifth region, 3bp deletion (mature form)
aacaaauucagaaaugaagga

SEQ ID NO: 115 - RNA, 23 nt, Artificial Sequence
  fourth region + Linker + fifth region, 2bp deletion (mature form)
aacaaauucaugaaaaugaagga

SEQ ID NO: 116 - RNA, 25 nt, Artificial Sequence
  fourth region + Linker + fifth region, 1bp deletion (mature form)
aacaaauucauugaaaaaugaagga

SEQ ID NO: 117 - RNA, 27 nt, Artificial Sequence
  fourth region + Linker + fifth region (mature form)
aacaaauucauuugaaagaaugaagga

SEQ ID NO: 118 - RNA, 120 nt, Artificial Sequence
  engineered tracrRNA(mature form, 20nt deletion in the first region)
accgcuucaccaaaagcugucccuuaggggauuagaacuugagugaaggugggcugcuugcaucagccuaaugucgagaagugcuuucuucggaaaguaacccucgaaacaaauucauuu

SEQ ID NO: 119 - RNA, 121 nt, Artificial Sequence
  engineered tracrRNA(mature form, 19nt deletion in the first region)
aaccgcuucaccaaaagcugucccuuaggggauuagaacuugagugaaggugggcugcuugcaucagccuaaugucgagaagugcuuucuucggaaaguaacccucgaaacaaauucauuu

SEQ ID NO: 120 - RNA, 122 nt, Artificial Sequence
  engineered tracrRNA(mature form, 18nt deletion in the first region)
gaaccgcuucaccaaaagcugucccuuaggggauuagaacuugagugaaggugggcugcuugcaucagccuaaugucgagaagugcuuucuucggaaaguaacccucgaaacaaauucauuu

SEQ ID NO: 121 - RNA, 123 nt, Artificial Sequence
  engineered tracrRNA(mature form, 17nt deletion in the first region)
agaaccgcuucaccaaaagcugucccuuaggggauuagaacuugagugaaggugggcugcuugcaucagccuaaugucgagaagugcuuucuucggaaaguaacccucgaaacaaauucauuu

SEQ ID NO: 122 - RNA, 124 nt, Artificial Sequence
  engineered tracrRNA(mature form, 16nt deletion in the first region)
gagaaccgcuucaccaaaagcugucccuuaggggauuagaacuugagugaaggugggcugcuugcaucagccuaaugucgagaagugcuuucuucggaaaguaacccucgaaacaaauucauuu

SEQ ID NO: 123 - RNA, 125 nt, Artificial Sequence
  engineered tracrRNA(mature form, 15nt deletion in the first region)
ggagaaccgcuucaccaaaagcugucccuuaggggauuagaacuugagugaaggugggcugcuugcaucagccuaaugucgagaagugcuuucuucggaaaguaacccucgaaacaaauucauuu

SEQ ID NO: 124 - RNA, 126 nt, Artificial Sequence
  engineered tracrRNA(mature form, 14nt deletion in the first region)
uggagaaccgcuucaccaaaagcugucccuuaggggauuagaacuugagugaaggugggcugcuugcaucagccuaaugucgagaagugcuuucuucggaaaguaacccucgaaacaaauucauuu

SEQ ID NO: 125 - RNA, 127 nt, Artificial Sequence
  engineered tracrRNA(mature form, 13nt deletion in the first region)
guggagaaccgcuucaccaaaagcugucccuuaggggauuagaacuugagugaaggugggcugcuugcaucagccuaaugucgagaagugcuuucuucggaaaguaacccucgaaacaaauucauuu

SEQ ID NO: 126 - RNA, 128 nt, Artificial Sequence
  engineered tracrRNA(mature form, 12nt deletion in the first region)
aguggagaaccgcuucaccaaaagcugucccuuaggggauuagaacuugagugaaggugggcugcuugcaucagccuaaugucgagaagugcuuucuucggaaaguaacccucgaaacaaauucauuu

SEQ ID NO: 127 - RNA, 129 nt, Artificial Sequence
  engineered tracrRNA(mature form, 11nt deletion in the first region)
aaguggagaaccgcuucaccaaaagcugucccuuaggggauuagaacuugagugaaggugggcugcuugcaucagccuaaugucgagaagugcuuucuucggaaaguaacccucgaaacaaauucauuu

SEQ ID NO: 128 - RNA, 130 nt, Artificial Sequence
  engineered tracrRNA(mature form, 10nt deletion in the first region)
aaaguggagaaccgcuucaccaaaagcugucccuuaggggauuagaacuugagugaaggugggcugcuugcaucagccuaaugucgagaagugcuuucuucggaaaguaacccucgaaacaaauucauuu

SEQ ID NO: 129 - RNA, 131 nt, Artificial Sequence
  engineered tracrRNA(mature form, 9nt deletion in the first region)
uaaaguggagaaccgcuucaccaaaagcugucccuuaggggauuagaacuugagugaaggugggcugcuugcaucagccuaaugucgagaagugcuuucuucggaaaguaacccucgaaacaaauucauuu

SEQ ID NO: 130 - RNA, 132 nt, Artificial Sequence
  engineered tracrRNA(mature form, 8nt deletion in the first region)
auaaaguggagaaccgcuucaccaaaagcugucccuuaggggauuagaacuugagugaaggugggcugcuugcaucagccuaaugucgagaagugcuuucuucggaaaguaacccucgaaacaaauucauuu

SEQ ID NO: 131 - RNA, 133 nt, Artificial Sequence
  engineered tracrRNA(mature form, 7nt deletion in the first region)
gauaaaguggagaaccgcuucaccaaaagcugucccuuaggggauuagaacuugagugaaggugggcugcuugcaucagccuaaugucgagaagugcuuucuucggaaaguaacccucgaaacaaauucauuu

SEQ ID NO: 132 - RNA, 134 nt, Artificial Sequence
  engineered tracrRNA(mature form, 6nt deletion in the first region)
ugauaaaguggagaaccgcuucaccaaaagcugucccuuaggggauuagaacuugagugaaggugggcugcuugcaucagccuaaugucgagaagugcuuucuucggaaaguaacccucgaaacaaauucauuu

SEQ ID NO: 133 - RNA, 135 nt, Artificial Sequence
  engineered tracrRNA(mature form, 5nt deletion in the first region)
cugauaaaguggagaaccgcuucaccaaaagcugucccuuaggggauuagaacuugagugaaggugggcugcuugcaucagccuaaugucgagaagugcuuucuucggaaaguaacccucgaaacaaauucauuu

SEQ ID NO: 134 - RNA, 136 nt, Artificial Sequence
  engineered tracrRNA(mature form, 4nt deletion in the first region)
acugauaaaguggagaaccgcuucaccaaaagcugucccuuaggggauuagaacuugagugaaggugggcugcuugcaucagccuaaugucgagaagugcuuucuucggaaaguaacccucgaaacaaauucauuu

SEQ ID NO: 135 - RNA, 137 nt, Artificial Sequence
  engineered tracrRNA(mature form, 3nt deletion in the first region)
cacugauaaaguggagaaccgcuucaccaaaagcugucccuuaggggauuagaacuugagugaaggugggcugcuugcaucagccuaaugucgagaagugcuuucuucggaaaguaacccucgaaacaaauucauuu

SEQ ID NO: 136 - RNA, 138 nt, Artificial Sequence
  engineered tracrRNA(mature form, 2nt deletion in the first region)
ucacugauaaaguggagaaccgcuucaccaaaagcugucccuuaggggauuagaacuugagugaaggugggcugcuugcaucagccuaaugucgagaagugcuuucuucggaaaguaacccucgaaacaaauucauuu

SEQ ID NO: 137 - RNA, 139 nt, Artificial Sequence
  engineered tracrRNA(mature form, 1nt deletion in the first region)
uucacugauaaaguggagaaccgcuucaccaaaagcugucccuuaggggauuagaacuugagugaaggugggcugcuugcaucagccuaaugucgagaagugcuuucuucggaaaguaacccucgaaacaaauucauuu

SEQ ID NO: 138 - RNA, 117 nt, Artificial Sequence
  engineered tracrRNA(mature form, 10bp deletion in the second region)
cuucacugauaaaguggagaaccgcuucaccauuagugagugaaggugggcugcuugcaucagccuaaugucgagaagugcuuucuucggaaaguaacccucgaaacaaauucauuu

SEQ ID NO: 139 - RNA, 119 nt, Artificial Sequence
  engineered tracrRNA(mature form, 9bp deletion in the second region)
cuucacugauaaaguggagaaccgcuucaccaauuaguugagugaaggugggcugcuugcaucagccuaaugucgagaagugcuuucuucggaaaguaacccucgaaacaaauucauuu

SEQ ID NO: 140 - RNA, 122 nt, Artificial Sequence
  engineered tracrRNA(mature form, 8bp deletion in the second region)
cuucacugauaaaguggagaaccgcuucaccaaauuagacuugagugaaggugggcugcuugcaucagccuaaugucgagaagugcuuucuucggaaaguaacccucgaaacaaauucauuu

SEQ ID NO: 141 - RNA, 125 nt, Artificial Sequence
  engineered tracrRNA(mature form, 7bp deletion in the second region)
cuucacugauaaaguggagaaccgcuucaccaaaaguuagaacuugagugaaggugggcugcuugcaucagccuaaugucgagaagugcuuucuucggaaaguaacccucgaaacaaauucauuu

SEQ ID NO: 142 - RNA, 127 nt, Artificial Sequence
  engineered tracrRNA(mature form, 6bp deletion in the second region)
cuucacugauaaaguggagaaccgcuucaccaaaagcuuaggaacuugagugaaggugggcugcuugcaucagccuaaugucgagaagugcuuucuucggaaaguaacccucgaaacaaauucauuu

SEQ ID NO: 143 - RNA, 129 nt, Artificial Sequence
  engineered tracrRNA(mature form, 5bp deletion in the second region)
cuucacugauaaaguggagaaccgcuucaccaaaagcuuuagagaacuugagugaaggugggcugcuugcaucagccuaaugucgagaagugcuuucuucggaaaguaacccucgaaacaaauucauuu

SEQ ID NO: 144 - RNA, 132 nt, Artificial Sequence
  engineered tracrRNA(mature form, 4bp deletion in the second region)
cuucacugauaaaguggagaaccgcuucaccaaaagcuguuaguuagaacuugagugaaggugggcugcuugcaucagccuaaugucgagaagugcuuucuucggaaaguaacccucgaaacaaauucauuu

SEQ ID NO: 145 - RNA, 131 nt, Artificial Sequence
  engineered tracrRNA(mature form, 4bp+1nt deletion in the second region)
cuucacugauaaaguggagaaccgcuucaccaaaagcuguuaguagaacuugagugaaggugggcugcuugcaucagccuaaugucgagaagugcuuucuucggaaaguaacccucgaaacaaauucauuu

SEQ ID NO: 146 - RNA, 134 nt, Artificial Sequence
  engineered tracrRNA(mature form, 3bp deletion in the second region)
cuucacugauaaaguggagaaccgcuucaccaaaagcuguuuagauuagaacuugagugaaggugggcugcuugcaucagccuaaugucgagaagugcuuucuucggaaaguaacccucgaaacaaauucauuu

SEQ ID NO: 147 - RNA, 136 nt, Artificial Sequence
  engineered tracrRNA(mature form, 2bp deletion in the second region)
cuucacugauaaaguggagaaccgcuucaccaaaagcugucuuaggauuagaacuugagugaaggugggcugcuugcaucagccuaaugucgagaagugcuuucuucggaaaguaacccucgaaacaaauucauuu

SEQ ID NO: 148 - RNA, 138 nt, Artificial Sequence
  engineered tracrRNA(mature form, 1bp deletion in the second region)
cuucacugauaaaguggagaaccgcuucaccaaaagcuguccuuagggauuagaacuugagugaaggugggcugcuugcaucagccuaaugucgagaagugcuuucuucggaaaguaacccucgaaacaaauucauuu

SEQ ID NO: 149 - RNA, 133 nt, Artificial Sequence
  engineered tracrRNA(mature form, 7nt deletion in the fourth region)
cuucacugauaaaguggagaaccgcuucaccaaaagcugucccuuaggggauuagaacuugagugaaggugggcugcuugcaucagccuaaugucgagaagugcuuucuucggaaaguaacccucgaaacaaa

SEQ ID NO: 150 - RNA, 134 nt, Artificial Sequence
  engineered tracrRNA(mature form, 6nt deletion in the fourth region)
cuucacugauaaaguggagaaccgcuucaccaaaagcugucccuuaggggauuagaacuugagugaaggugggcugcuugcaucagccuaaugucgagaagugcuuucuucggaaaguaacccucgaaacaaau

SEQ ID NO: 151 - RNA, 135 nt, Artificial Sequence
  engineered tracrRNA(mature form, 5nt deletion in the fourth region)
cuucacugauaaaguggagaaccgcuucaccaaaagcugucccuuaggggauuagaacuugagugaaggugggcugcuugcaucagccuaaugucgagaagugcuuucuucggaaaguaacccucgaaacaaauu

SEQ ID NO: 152 - RNA, 136 nt, Artificial Sequence
  engineered tracrRNA(mature form, 4nt deletion in the fourth region)
cuucacugauaaaguggagaaccgcuucaccaaaagcugucccuuaggggauuagaacuugagugaaggugggcugcuugcaucagccuaaugucgagaagugcuuucuucggaaaguaacccucgaaacaaauuc

SEQ ID NO: 153 - RNA, 137 nt, Artificial Sequence
  engineered tracrRNA(mature form, 3nt deletion in the fourth region)
cuucacugauaaaguggagaaccgcuucaccaaaagcugucccuuaggggauuagaacuugagugaaggugggcugcuugcaucagccuaaugucgagaagugcuuucuucggaaaguaacccucgaaacaaauuca

SEQ ID NO: 154 - RNA, 138 nt, Artificial Sequence
  engineered tracrRNA(mature form, 2nt deletion in the fourth region)
cuucacugauaaaguggagaaccgcuucaccaaaagcugucccuuaggggauuagaacuugagugaaggugggcugcuugcaucagccuaaugucgagaagugcuuucuucggaaaguaacccucgaaacaaauucau

SEQ ID NO: 155 - RNA, 139 nt, Artificial Sequence
  engineered tracrRNA(mature form, 1nt deletion in the fourth region)
cuucacugauaaaguggagaaccgcuucaccaaaagcugucccuuaggggauuagaacuugagugaaggugggcugcuugcaucagccuaaugucgagaagugcuuucuucggaaaguaacccucgaaacaaauucauu

SEQ ID NO: 156 - RNA, 97 nt, Artificial Sequence
  engineered tracrRNA(mature form, modified first region and modified second region)
accgcuucaccauuagugagugaaggugggcugcuugcaucagccuaaugucgagaagugcuuucuucggaaaguaacccucgaaacaaauucauuu

SEQ ID NO: 157 - RNA, 113 nt, Artificial Sequence
  engineered tracrRNA(mature form, modified first region and modified fourth and fifth region)
accgcuucaccaaaagcugucccuuaggggauuagaacuugagugaaggugggcugcuugcaucagccuaaugucgagaagugcuuucuucggaaaguaacccucgaaacaaa

SEQ ID NO: 158 - RNA, 110 nt, Artificial Sequence
  engineered tracrRNA(mature form, modified second region and modified fourth and fifth region)
cuucacugauaaaguggagaaccgcuucaccauuagugagugaaggugggcugcuugcaucagccuaaugucgagaagugcuuucuucggaaaguaacccucgaaacaaa

SEQ ID NO: 159 - RNA, 90 nt, Artificial Sequence
  engineered tracrRNA(mature form, modified first region, modified second region, modified fourth and fifth region)
accgcuucaccauuagugagugaaggugggcugcuugcaucagccuaaugucgagaagugcuuucuucggaaaguaacccucgaaacaaa

SEQ ID NO: 160 - RNA, 10 nt, Artificial Sequence
  engineered crRNA repeat(mature form, 7nt deletion in the fifth region)
ggaaugcaac

SEQ ID NO: 161 - RNA, 11 nt, Artificial Sequence
  engineered crRNA repeat(mature form, 6nt deletion in the fifth region)
aggaaugcaac

SEQ ID NO: 162 - RNA, 12 nt, Artificial Sequence
  engineered crRNA repeat(mature form, 5nt deletion in the fifth region)
aaggaaugcaac

SEQ ID NO: 163 - RNA, 13 nt, Artificial Sequence
  engineered crRNA repeat(mature form, 4nt deletion in the fifth region)
gaaggaaugcaac

SEQ ID NO: 164 - RNA, 14 nt, Artificial Sequence
  engineered crRNA repeat(mature form, 3nt deletion in the fifth region)
ugaaggaaugcaac

SEQ ID NO: 165 - RNA, 15 nt, Artificial Sequence
  engineered crRNA repeat(mature form, 2nt deletion in the fifth region)
augaaggaaugcaac

SEQ ID NO: 166 - RNA, 16 nt, Artificial Sequence
  engineered crRNA repeat(mature form, 1nt deletion in the fifth region)
aaugaaggaaugcaac

SEQ ID NO: 167 - RNA, 141 nt, Artificial Sequence
  engineered scaffold(mature form, 20nt deletion in the first region)
accgcuucaccaaaagcugucccuuaggggauuagaacuugagugaaggugggcugcuugcaucagccuaaugucgagaagugcuuucuucggaaaguaacccucgaaacaaauucauuugaaagaaugaaggaaugcaac

SEQ ID NO: 168 - RNA, 142 nt, Artificial Sequence
  engineered scaffold(mature form, 19nt deletion in the first region)
aaccgcuucaccaaaagcugucccuuaggggauuagaacuugagugaaggugggcugcuugcaucagccuaaugucgagaagugcuuucuucggaaaguaacccucgaaacaaauucauuugaaagaaugaaggaaugcaac

SEQ ID NO: 169 - RNA, 143 nt, Artificial Sequence
  engineered scaffold(mature form, 18nt deletion in the first region)
gaaccgcuucaccaaaagcugucccuuaggggauuagaacuugagugaaggugggcugcuugcaucagccuaaugucgagaagugcuuucuucggaaaguaacccucgaaacaaauucauuugaaagaaugaaggaaugcaac

SEQ ID NO: 170 - RNA, 144 nt, Artificial Sequence
  engineered scaffold(mature form, 17nt deletion in the first region)
agaaccgcuucaccaaaagcugucccuuaggggauuagaacuugagugaaggugggcugcuugcaucagccuaaugucgagaagugcuuucuucggaaaguaacccucgaaacaaauucauuugaaagaaugaaggaaugcaac

SEQ ID NO: 171 - RNA, 145 nt, Artificial Sequence
  engineered scaffold(mature form, 16nt deletion in the first region)
gagaaccgcuucaccaaaagcugucccuuaggggauuagaacuugagugaaggugggcugcuugcaucagccuaaugucgagaagugcuuucuucggaaaguaacccucgaaacaaauucauuugaaagaaugaaggaaugcaac

SEQ ID NO: 172 - RNA, 146 nt, Artificial Sequence
  engineered scaffold(mature form, 15nt deletion in the first region)
ggagaaccgcuucaccaaaagcugucccuuaggggauuagaacuugagugaaggugggcugcuugcaucagccuaaugucgagaagugcuuucuucggaaaguaacccucgaaacaaauucauuugaaagaaugaaggaaugcaac

SEQ ID NO: 173 - RNA, 147 nt, Artificial Sequence
  engineered scaffold(mature form, 14nt deletion in the first region)
uggagaaccgcuucaccaaaagcugucccuuaggggauuagaacuugagugaaggugggcugcuugcaucagccuaaugucgagaagugcuuucuucggaaaguaacccucgaaacaaauucauuugaaagaaugaaggaaugcaac

SEQ ID NO: 174 - RNA, 148 nt, Artificial Sequence
  engineered scaffold(mature form, 13nt deletion in the first region)
guggagaaccgcuucaccaaaagcugucccuuaggggauuagaacuugagugaaggugggcugcuugcaucagccuaaugucgagaagugcuuucuucggaaaguaacccucgaaacaaauucauuugaaagaaugaaggaaugcaac

SEQ ID NO: 175 - RNA, 149 nt, Artificial Sequence
  engineered scaffold(mature form, 12nt deletion in the first region)
aguggagaaccgcuucaccaaaagcugucccuuaggggauuagaacuugagugaaggugggcugcuugcaucagccuaaugucgagaagugcuuucuucggaaaguaacccucgaaacaaauucauuugaaagaaugaaggaaugcaac

SEQ ID NO: 176 - RNA, 150 nt, Artificial Sequence
  engineered scaffold(mature form, 11nt deletion in the first region)
aaguggagaaccgcuucaccaaaagcugucccuuaggggauuagaacuugagugaaggugggcugcuugcaucagccuaaugucgagaagugcuuucuucggaaaguaacccucgaaacaaauucauuugaaagaaugaaggaaugcaac

SEQ ID NO: 177 - RNA, 151 nt, Artificial Sequence
  engineered scaffold(mature form, 10nt deletion in the first region)
aaaguggagaaccgcuucaccaaaagcugucccuuaggggauuagaacuugagugaaggugggcugcuugcaucagccuaaugucgagaagugcuuucuucggaaaguaacccucgaaacaaauucauuugaaagaaugaaggaaugcaac

SEQ ID NO: 178 - RNA, 152 nt, Artificial Sequence
  engineered scaffold(mature form, 9nt deletion in the first region)
uaaaguggagaaccgcuucaccaaaagcugucccuuaggggauuagaacuugagugaaggugggcugcuugcaucagccuaaugucgagaagugcuuucuucggaaaguaacccucgaaacaaauucauuugaaagaaugaaggaaugcaac

SEQ ID NO: 179 - RNA, 153 nt, Artificial Sequence
  engineered scaffold(mature form, 8nt deletion in the first region)
auaaaguggagaaccgcuucaccaaaagcugucccuuaggggauuagaacuugagugaaggugggcugcuugcaucagccuaaugucgagaagugcuuucuucggaaaguaacccucgaaacaaauucauuugaaagaaugaaggaaugcaac

SEQ ID NO: 180 - RNA, 154 nt, Artificial Sequence
  engineered scaffold(mature form, 7nt deletion in the first region)
gauaaaguggagaaccgcuucaccaaaagcugucccuuaggggauuagaacuugagugaaggugggcugcuugcaucagccuaaugucgagaagugcuuucuucggaaaguaacccucgaaacaaauucauuugaaagaaugaaggaaugcaac

SEQ ID NO: 181 - RNA, 155 nt, Artificial Sequence
  engineered scaffold(mature form, 6nt deletion in the first region)
ugauaaaguggagaaccgcuucaccaaaagcugucccuuaggggauuagaacuugagugaaggugggcugcuugcaucagccuaaugucgagaagugcuuucuucggaaaguaacccucgaaacaaauucauuugaaagaaugaaggaaugcaac

SEQ ID NO: 182 - RNA, 156 nt, Artificial Sequence
  engineered scaffold(mature form, 5nt deletion in the first region)
cugauaaaguggagaaccgcuucaccaaaagcugucccuuaggggauuagaacuugagugaaggugggcugcuugcaucagccuaaugucgagaagugcuuucuucggaaaguaacccucgaaacaaauucauuugaaagaaugaaggaaugcaac

SEQ ID NO: 183 - RNA, 157 nt, Artificial Sequence
  engineered scaffold(mature form, 4nt deletion in the first region)
acugauaaaguggagaaccgcuucaccaaaagcugucccuuaggggauuagaacuugagugaaggugggcugcuugcaucagccuaaugucgagaagugcuuucuucggaaaguaacccucgaaacaaauucauuugaaagaaugaaggaaugcaac

SEQ ID NO: 184 - RNA, 158 nt, Artificial Sequence
  engineered scaffold(mature form, 3nt deletion in the first region)
cacugauaaaguggagaaccgcuucaccaaaagcugucccuuaggggauuagaacuugagugaaggugggcugcuugcaucagccuaaugucgagaagugcuuucuucggaaaguaacccucgaaacaaauucauuugaaagaaugaaggaaugcaac

SEQ ID NO: 185 - RNA, 159 nt, Artificial Sequence
  engineered scaffold(mature form, 2nt deletion in the first region)
ucacugauaaaguggagaaccgcuucaccaaaagcugucccuuaggggauuagaacuugagugaaggugggcugcuugcaucagccuaaugucgagaagugcuuucuucggaaaguaacccucgaaacaaauucauuugaaagaaugaaggaaugcaac

SEQ ID NO: 186 - RNA, 160 nt, Artificial Sequence
  engineered scaffold(mature form, 1nt deletion in the first region)
uucacugauaaaguggagaaccgcuucaccaaaagcugucccuuaggggauuagaacuugagugaaggugggcugcuugcaucagccuaaugucgagaagugcuuucuucggaaaguaacccucgaaacaaauucauuugaaagaaugaaggaaugcaac

SEQ ID NO: 187 - RNA, 138 nt, Artificial Sequence
  engineered scaffold(mature form, 11bp deletion in the second region)
cuucacugauaaaguggagaaccgcuucaccauuagugagugaaggugggcugcuugcaucagccuaaugucgagaagugcuuucuucggaaaguaacccucgaaacaaauucauuugaaagaaugaaggaaugcaac

SEQ ID NO: 188 - RNA, 140 nt, Artificial Sequence
  engineered scaffold(mature form, 10bp deletion in the second region)
cuucacugauaaaguggagaaccgcuucaccaauuaguugagugaaggugggcugcuugcaucagccuaaugucgagaagugcuuucuucggaaaguaacccucgaaacaaauucauuugaaagaaugaaggaaugcaac

SEQ ID NO: 189 - RNA, 142 nt, Artificial Sequence
  engineered scaffold(mature form, 9bp deletion in the second region)
cuucacugauaaaguggagaaccgcuucaccaaauuagcuugagugaaggugggcugcuugcaucagccuaaugucgagaagugcuuucuucggaaaguaacccucgaaacaaauucauuugaaagaaugaaggaaugcaac

SEQ ID NO: 190 - RNA, 144 nt, Artificial Sequence
  engineered scaffold(mature form, 8bp deletion in the second region)
cuucacugauaaaguggagaaccgcuucaccaaaauuagacuugagugaaggugggcugcuugcaucagccuaaugucgagaagugcuuucuucggaaaguaacccucgaaacaaauucauuugaaagaaugaaggaaugcaac

SEQ ID NO: 191 - RNA, 146 nt, Artificial Sequence
  engineered scaffold(mature form, 7bp deletion in the second region)
cuucacugauaaaguggagaaccgcuucaccaaaaguuagaacuugagugaaggugggcugcuugcaucagccuaaugucgagaagugcuuucuucggaaaguaacccucgaaacaaauucauuugaaagaaugaaggaaugcaac

SEQ ID NO: 192 - RNA, 148 nt, Artificial Sequence
  engineered scaffold(mature form, 6bp deletion in the second region)
cuucacugauaaaguggagaaccgcuucaccaaaagcuuaggaacuugagugaaggugggcugcuugcaucagccuaaugucgagaagugcuuucuucggaaaguaacccucgaaacaaauucauuugaaagaaugaaggaaugcaac

SEQ ID NO: 193 - RNA, 150 nt, Artificial Sequence
  engineered scaffold(mature form, 5bp deletion in the second region)
cuucacugauaaaguggagaaccgcuucaccaaaagcuuuagagaacuugagugaaggugggcugcuugcaucagccuaaugucgagaagugcuuucuucggaaaguaacccucgaaacaaauucauuugaaagaaugaaggaaugcaac

SEQ ID NO: 194 - RNA, 152 nt, Artificial Sequence
  engineered scaffold(mature form, 4bp deletion in the second region)
cuucacugauaaaguggagaaccgcuucaccaaaagcuguuaguagaacuugagugaaggugggcugcuugcaucagccuaaugucgagaagugcuuucuucggaaaguaacccucgaaacaaauucauuugaaagaaugaaggaaugcaac

SEQ ID NO: 195 - RNA, 153 nt, Artificial Sequence
  engineered scaffold(mature form, 4bp+1nt deletion in the second region)
cuucacugauaaaguggagaaccgcuucaccaaaagcuguuaguuagaacuugagugaaggugggcugcuugcaucagccuaaugucgagaagugcuuucuucggaaaguaacccucgaaacaaauucauuugaaagaaugaaggaaugcaac

SEQ ID NO: 196 - RNA, 155 nt, Artificial Sequence
  engineered scaffold(mature form, 3bp deletion in the second region)
cuucacugauaaaguggagaaccgcuucaccaaaagcuguuuagauuagaacuugagugaaggugggcugcuugcaucagccuaaugucgagaagugcuuucuucggaaaguaacccucgaaacaaauucauuugaaagaaugaaggaaugcaac

SEQ ID NO: 197 - RNA, 157 nt, Artificial Sequence
  engineered scaffold(mature form, 2bp deletion in the second region)
cuucacugauaaaguggagaaccgcuucaccaaaagcugucuuaggauuagaacuugagugaaggugggcugcuugcaucagccuaaugucgagaagugcuuucuucggaaaguaacccucgaaacaaauucauuugaaagaaugaaggaaugcaac

SEQ ID NO: 198 - RNA, 159 nt, Artificial Sequence
  engineered scaffold(mature form, 1bp deletion in the second region)
cuucacugauaaaguggagaaccgcuucaccaaaagcuguccuuagggauuagaacuugagugaaggugggcugcuugcaucagccuaaugucgagaagugcuuucuucggaaaguaacccucgaaacaaauucauuugaaagaaugaaggaaugcaac

SEQ ID NO: 199 - RNA, 147 nt, Artificial Sequence
  engineered scaffold(mature form, 7bp deletion in the fourth and fifth region)
cuucacugauaaaguggagaaccgcuucaccaaaagcugucccuuaggggauuagaacuugagugaaggugggcugcuugcaucagccuaaugucgagaagugcuuucuucggaaaguaacccucgaaacaaagaaaggaaugcaac

SEQ ID NO: 200 - RNA, 149 nt, Artificial Sequence
  engineered scaffold(mature form, 6bp deletion in the fourth and fifth region)
cuucacugauaaaguggagaaccgcuucaccaaaagcugucccuuaggggauuagaacuugagugaaggugggcugcuugcaucagccuaaugucgagaagugcuuucuucggaaaguaacccucgaaacaaaugaaaaggaaugcaac

SEQ ID NO: 201 - RNA, 151 nt, Artificial Sequence
  engineered scaffold(mature form, 5bp deletion in the fourth and fifth region)
cuucacugauaaaguggagaaccgcuucaccaaaagcugucccuuaggggauuagaacuugagugaaggugggcugcuugcaucagccuaaugucgagaagugcuuucuucggaaaguaacccucgaaacaaauugaaaaaggaaugcaac

SEQ ID NO: 202 - RNA, 153 nt, Artificial Sequence
  engineered scaffold(mature form, 4bp deletion in the fourth and fifth region)
cuucacugauaaaguggagaaccgcuucaccaaaagcugucccuuaggggauuagaacuugagugaaggugggcugcuugcaucagccuaaugucgagaagugcuuucuucggaaaguaacccucgaaacaaauucgaaagaaggaaugcaac

SEQ ID NO: 203 - RNA, 155 nt, Artificial Sequence
  engineered scaffold(mature form, 3bp deletion in the fourth and fifth region)
cuucacugauaaaguggagaaccgcuucaccaaaagcugucccuuaggggauuagaacuugagugaaggugggcugcuugcaucagccuaaugucgagaagugcuuucuucggaaaguaacccucgaaacaaauucagaaaugaaggaaugcaac

SEQ ID NO: 204 - RNA, 157 nt, Artificial Sequence
  engineered scaffold(mature form, 2bp deletion in the fourth and fifth region)
cuucacugauaaaguggagaaccgcuucaccaaaagcugucccuuaggggauuagaacuugagugaaggugggcugcuugcaucagccuaaugucgagaagugcuuucuucggaaaguaacccucgaaacaaauucaugaaaaugaaggaaugcaac

SEQ ID NO: 205 - RNA, 159 nt, Artificial Sequence
  engineered scaffold(mature form, 1bp deletion in the fourth and fifth region)
cuucacugauaaaguggagaaccgcuucaccaaaagcugucccuuaggggauuagaacuugagugaaggugggcugcuugcaucagccuaaugucgagaagugcuuucuucggaaaguaacccucgaaacaaauucauugaaaaaugaaggaaugcaac

SEQ ID NO: 206 - RNA, 118 nt, Artificial Sequence
  engineered scaffold(mature form, modified first and second region)
accgcuucaccauuagugagugaaggugggcugcuugcaucagccuaaugucgagaagugcuuucuucggaaaguaacccucgaaacaaauucauuugaaagaaugaaggaaugcaac

SEQ ID NO: 207 - RNA, 127 nt, Artificial Sequence
  engineered scaffold(mature form, modified first, fourth and fifth region)
accgcuucaccaaaagcugucccuuaggggauuagaacuugagugaaggugggcugcuugcaucagccuaaugucgagaagugcuuucuucggaaaguaacccucgaaacaaagaaaggaaugcaac

SEQ ID NO: 208 - RNA, 124 nt, Artificial Sequence
  engineered scaffold(mature form, modified second, fourth and fifth region)
cuucacugauaaaguggagaaccgcuucaccauuagugagugaaggugggcugcuugcaucagccuaaugucgagaagugcuuucuucggaaaguaacccucgaaacaaagaaaggaaugcaac

SEQ ID NO: 209 - RNA, 104 nt, Artificial Sequence
  engineered scaffold(mature form, modified first, second, fourth and fifth region)
accgcuucaccauuagugagugaaggugggcugcuugcaucagccuaaugucgagaagugcuuucuucggaaaguaacccucgaaacaaagaaaggaaugcaac

SEQ ID NO: 210 - RNA, 189 nt, Artificial Sequence
  sgRNA(mature form, 1nt deletion in the first region)
uucacugauaaaguggagaaccgcuucaccaaaagcugucccuuaggggauuagaacuugagugaaggugggcugcuugcaucagccuaaugucgagaagugcuuucuucggaaaguaacccucgaaacaaauucauuugaaagaaugaaggaaugcaacnnnnnnnnnnnnnnnnnnnnuuuuauuuu

SEQ ID NO: 211 - RNA, 188 nt, Artificial Sequence
  sgRNA(mature form, 2nt deletion in the first region)
ucacugauaaaguggagaaccgcuucaccaaaagcugucccuuaggggauuagaacuugagugaaggugggcugcuugcaucagccuaaugucgagaagugcuuucuucggaaaguaacccucgaaacaaauucauuugaaagaaugaaggaaugcaacnnnnnnnnnnnnnnnnnnnnuuuuauuuu

SEQ ID NO: 212 - RNA, 187 nt, Artificial Sequence
  sgRNA(mature form, 3nt deletion in the first region)
cacugauaaaguggagaaccgcuucaccaaaagcugucccuuaggggauuagaacuugagugaaggugggcugcuugcaucagccuaaugucgagaagugcuuucuucggaaaguaacccucgaaacaaauucauuugaaagaaugaaggaaugcaacnnnnnnnnnnnnnnnnnnnnuuuuauuuu

SEQ ID NO: 213 - RNA, 186 nt, Artificial Sequence
  sgRNA(mature form, 4nt deletion in the first region)
acugauaaaguggagaaccgcuucaccaaaagcugucccuuaggggauuagaacuugagugaaggugggcugcuugcaucagccuaaugucgagaagugcuuucuucggaaaguaacccucgaaacaaauucauuugaaagaaugaaggaaugcaacnnnnnnnnnnnnnnnnnnnnuuuuauuuu

SEQ ID NO: 214 - RNA, 185 nt, Artificial Sequence
  sgRNA(mature form, 5nt deletion in the first region)
cugauaaaguggagaaccgcuucaccaaaagcugucccuuaggggauuagaacuugagugaaggugggcugcuugcaucagccuaaugucgagaagugcuuucuucggaaaguaacccucgaaacaaauucauuugaaagaaugaaggaaugcaacnnnnnnnnnnnnnnnnnnnnuuuuauuuu

SEQ ID NO: 215 - RNA, 184 nt, Artificial Sequence
  sgRNA(mature form, 6nt deletion in the first region)
ugauaaaguggagaaccgcuucaccaaaagcugucccuuaggggauuagaacuugagugaaggugggcugcuugcaucagccuaaugucgagaagugcuuucuucggaaaguaacccucgaaacaaauucauuugaaagaaugaaggaaugcaacnnnnnnnnnnnnnnnnnnnnuuuuauuuu

SEQ ID NO: 216 - RNA, 183 nt, Artificial Sequence
  sgRNA(mature form, 7nt deletion in the first region)
gauaaaguggagaaccgcuucaccaaaagcugucccuuaggggauuagaacuugagugaaggugggcugcuugcaucagccuaaugucgagaagugcuuucuucggaaaguaacccucgaaacaaauucauuugaaagaaugaaggaaugcaacnnnnnnnnnnnnnnnnnnnnuuuuauuuu

SEQ ID NO: 217 - RNA, 182 nt, Artificial Sequence
  sgRNA(mature form, 8nt deletion in the first region)
auaaaguggagaaccgcuucaccaaaagcugucccuuaggggauuagaacuugagugaaggugggcugcuugcaucagccuaaugucgagaagugcuuucuucggaaaguaacccucgaaacaaauucauuugaaagaaugaaggaaugcaacnnnnnnnnnnnnnnnnnnnnuuuuauuuu

SEQ ID NO: 218 - RNA, 181 nt, Artificial Sequence
  sgRNA(mature form, 9nt deletion in the first region)
uaaaguggagaaccgcuucaccaaaagcugucccuuaggggauuagaacuugagugaaggugggcugcuugcaucagccuaaugucgagaagugcuuucuucggaaaguaacccucgaaacaaauucauuugaaagaaugaaggaaugcaacnnnnnnnnnnnnnnnnnnnnuuuuauuuu

SEQ ID NO: 219 - RNA, 180 nt, Artificial Sequence
  sgRNA(mature form, 10nt deletion in the first region)
aaaguggagaaccgcuucaccaaaagcugucccuuaggggauuagaacuugagugaaggugggcugcuugcaucagccuaaugucgagaagugcuuucuucggaaaguaacccucgaaacaaauucauuugaaagaaugaaggaaugcaacnnnnnnnnnnnnnnnnnnnnuuuuauuuu

SEQ ID NO: 220 - RNA, 179 nt, Artificial Sequence
  sgRNA(mature form, 11nt deletion in the first region)
aaguggagaaccgcuucaccaaaagcugucccuuaggggauuagaacuugagugaaggugggcugcuugcaucagccuaaugucgagaagugcuuucuucggaaaguaacccucgaaacaaauucauuugaaagaaugaaggaaugcaacnnnnnnnnnnnnnnnnnnnnuuuuauuuu

SEQ ID NO: 221 - RNA, 170 nt, Artificial Sequence
  sgRNA(mature form, 12nt deletion in the first region)
aguggagaaccgcuucaccaaaagcugucccuuaggggauuagaacuugagugaaggugggcugcuugcaucagccuaaugucgagaagugcuuucuucggaaaguaacccucgaaacaaauucauuugaaagaaugaaggaaugcaacnnnnnnnnnnnnnnnnnnnnu

SEQ ID NO: 222 - RNA, 168 nt, Artificial Sequence
  sgRNA(mature form, 13nt deletion in the first region)
guggagaaccgcuucaccaaaagcugucccuuaggggauuagaacuugagugaaggugggcugcuugcaucagccuaaugucgagaagugcuuucuucggaaaguaacccucgaaacaaauucauuugaaagaaugaaggaaugcaacnnnnnnnnnnnnnnnnnnnn

SEQ ID NO: 223 - RNA, 167 nt, Artificial Sequence
  sgRNA(mature form, 14nt deletion in the first region)
uggagaaccgcuucaccaaaagcugucccuuaggggauuagaacuugagugaaggugggcugcuugcaucagccuaaugucgagaagugcuuucuucggaaaguaacccucgaaacaaauucauuugaaagaaugaaggaaugcaacnnnnnnnnnnnnnnnnnnnn

SEQ ID NO: 224 - RNA, 166 nt, Artificial Sequence
  sgRNA(mature form, 15nt deletion in the first region)
ggagaaccgcuucaccaaaagcugucccuuaggggauuagaacuugagugaaggugggcugcuugcaucagccuaaugucgagaagugcuuucuucggaaaguaacccucgaaacaaauucauuugaaagaaugaaggaaugcaacnnnnnnnnnnnnnnnnnnnn

SEQ ID NO: 225 - RNA, 165 nt, Artificial Sequence
  sgRNA(mature form, 16nt deletion in the first region)
gagaaccgcuucaccaaaagcugucccuuaggggauuagaacuugagugaaggugggcugcuugcaucagccuaaugucgagaagugcuuucuucggaaaguaacccucgaaacaaauucauuugaaagaaugaaggaaugcaacnnnnnnnnnnnnnnnnnnnn

SEQ ID NO: 226 - RNA, 164 nt, Artificial Sequence
  sgRNA(mature form, 17nt deletion in the first region)
agaaccgcuucaccaaaagcugucccuuaggggauuagaacuugagugaaggugggcugcuugcaucagccuaaugucgagaagugcuuucuucggaaaguaacccucgaaacaaauucauuugaaagaaugaaggaaugcaacnnnnnnnnnnnnnnnnnnnn

SEQ ID NO: 227 - RNA, 163 nt, Artificial Sequence
  sgRNA(mature form, 18nt deletion in the first region)
gaaccgcuucaccaaaagcugucccuuaggggauuagaacuugagugaaggugggcugcuugcaucagccuaaugucgagaagugcuuucuucggaaaguaacccucgaaacaaauucauuugaaagaaugaaggaaugcaacnnnnnnnnnnnnnnnnnnnn

SEQ ID NO: 228 - RNA, 162 nt, Artificial Sequence
  sgRNA(mature form, 19nt deletion in the first region)
aaccgcuucaccaaaagcugucccuuaggggauuagaacuugagugaaggugggcugcuugcaucagccuaaugucgagaagugcuuucuucggaaaguaacccucgaaacaaauucauuugaaagaaugaaggaaugcaacnnnnnnnnnnnnnnnnnnnn

SEQ ID NO: 229 - RNA, 161 nt, Artificial Sequence
  sgRNA(mature form, 20nt deletion in the first region)
accgcuucaccaaaagcugucccuuaggggauuagaacuugagugaaggugggcugcuugcaucagccuaaugucgagaagugcuuucuucggaaaguaacccucgaaacaaauucauuugaaagaaugaaggaaugcaacnnnnnnnnnnnnnnnnnnnn

SEQ ID NO: 230 - RNA, 179 nt, Artificial Sequence
  sgRNA(mature form, 1bp deletion in the second region)
cuucacugauaaaguggagaaccgcuucaccaaaagcuguccuuagggauuagaacuugagugaaggugggcugcuugcaucagccuaaugucgagaagugcuuucuucggaaaguaacccucgaaacaaauucauuugaaagaaugaaggaaugcaacnnnnnnnnnnnnnnnnnnnn

SEQ ID NO: 231 - RNA, 177 nt, Artificial Sequence
  sgRNA(mature form, 2bp deletion in the second region)
cuucacugauaaaguggagaaccgcuucaccaaaagcugucuuaggauuagaacuugagugaaggugggcugcuugcaucagccuaaugucgagaagugcuuucuucggaaaguaacccucgaaacaaauucauuugaaagaaugaaggaaugcaacnnnnnnnnnnnnnnnnnnnn

SEQ ID NO: 232 - RNA, 175 nt, Artificial Sequence
  sgRNA(mature form, 3bp deletion in the second region)
cuucacugauaaaguggagaaccgcuucaccaaaagcuguuuagauuagaacuugagugaaggugggcugcuugcaucagccuaaugucgagaagugcuuucuucggaaaguaacccucgaaacaaauucauuugaaagaaugaaggaaugcaacnnnnnnnnnnnnnnnnnnnn

SEQ ID NO: 233 - RNA, 173 nt, Artificial Sequence
  sgRNA(mature form, 4bp+1nt deletion in the second region)
cuucacugauaaaguggagaaccgcuucaccaaaagcuguuaguuagaacuugagugaaggugggcugcuugcaucagccuaaugucgagaagugcuuucuucggaaaguaacccucgaaacaaauucauuugaaagaaugaaggaaugcaacnnnnnnnnnnnnnnnnnnnn

SEQ ID NO: 234 - RNA, 172 nt, Artificial Sequence
  sgRNA(mature form, 4bp deletion in the second region)
cuucacugauaaaguggagaaccgcuucaccaaaagcuguuaguagaacuugagugaaggugggcugcuugcaucagccuaaugucgagaagugcuuucuucggaaaguaacccucgaaacaaauucauuugaaagaaugaaggaaugcaacnnnnnnnnnnnnnnnnnnnn

SEQ ID NO: 235 - RNA, 170 nt, Artificial Sequence
  sgRNA(mature form, 5bp deletion in the second region)
cuucacugauaaaguggagaaccgcuucaccaaaagcuuuagagaacuugagugaaggugggcugcuugcaucagccuaaugucgagaagugcuuucuucggaaaguaacccucgaaacaaauucauuugaaagaaugaaggaaugcaacnnnnnnnnnnnnnnnnnnnn

SEQ ID NO: 236 - RNA, 168 nt, Artificial Sequence
  sgRNA(mature form, 6bp deletion in the second region)
cuucacugauaaaguggagaaccgcuucaccaaaagcuuaggaacuugagugaaggugggcugcuugcaucagccuaaugucgagaagugcuuucuucggaaaguaacccucgaaacaaauucauuugaaagaaugaaggaaugcaacnnnnnnnnnnnnnnnnnnnn

SEQ ID NO: 237 - RNA, 166 nt, Artificial Sequence
  sgRNA(mature form, 7bp deletion in the second region)
cuucacugauaaaguggagaaccgcuucaccaaaaguuagaacuugagugaaggugggcugcuugcaucagccuaaugucgagaagugcuuucuucggaaaguaacccucgaaacaaauucauuugaaagaaugaaggaaugcaacnnnnnnnnnnnnnnnnnnnn

SEQ ID NO: 238 - RNA, 164 nt, Artificial Sequence
  sgRNA(mature form, 8bp deletion in the second region)
cuucacugauaaaguggagaaccgcuucaccaaaauuagacuugagugaaggugggcugcuugcaucagccuaaugucgagaagugcuuucuucggaaaguaacccucgaaacaaauucauuugaaagaaugaaggaaugcaacnnnnnnnnnnnnnnnnnnnn

SEQ ID NO: 239 - RNA, 162 nt, Artificial Sequence
  sgRNA(mature form, 9bp deletion in the second region)
cuucacugauaaaguggagaaccgcuucaccaaauuagcuugagugaaggugggcugcuugcaucagccuaaugucgagaagugcuuucuucggaaaguaacccucgaaacaaauucauuugaaagaaugaaggaaugcaacnnnnnnnnnnnnnnnnnnnn

SEQ ID NO: 240 - RNA, 160 nt, Artificial Sequence
  sgRNA(mature form, 10bp deletion in the second region)
cuucacugauaaaguggagaaccgcuucaccaauuaguugagugaaggugggcugcuugcaucagccuaaugucgagaagugcuuucuucggaaaguaacccucgaaacaaauucauuugaaagaaugaaggaaugcaacnnnnnnnnnnnnnnnnnnnn

SEQ ID NO: 241 - RNA, 167 nt, Artificial Sequence
  sgRNA(mature form, 11bp deletion in the second region)
cuucacugauaaaguggagaaccgcuucaccauuagugagugaaggugggcugcuugcaucagccuaaugucgagaagugcuuucuucggaaaguaacccucgaaacaaauucauuugaaagaaugaaggaaugcaacnnnnnnnnnnnnnnnnnnnnuuuuauuuu

SEQ ID NO: 242 - RNA, 179 nt, Artificial Sequence
  sgRNA(mature form, 1bp deletion in the fourth and fifth region)
cuucacugauaaaguggagaaccgcuucaccaaaagcugucccuuaggggauuagaacuugagugaaggugggcugcuugcaucagccuaaugucgagaagugcuuucuucggaaaguaacccucgaaacaaauucauugaaaaaugaaggaaugcaacnnnnnnnnnnnnnnnnnnnn

SEQ ID NO: 243 - RNA, 177 nt, Artificial Sequence
  sgRNA(mature form, 2bp deletion in the fourth and fifth region)
cuucacugauaaaguggagaaccgcuucaccaaaagcugucccuuaggggauuagaacuugagugaaggugggcugcuugcaucagccuaaugucgagaagugcuuucuucggaaaguaacccucgaaacaaauucaugaaaaugaaggaaugcaacnnnnnnnnnnnnnnnnnnnn

SEQ ID NO: 244 - RNA, 175 nt, Artificial Sequence
  sgRNA(mature form, 3bp deletion in the fourth and fifth region)
cuucacugauaaaguggagaaccgcuucaccaaaagcugucccuuaggggauuagaacuugagugaaggugggcugcuugcaucagccuaaugucgagaagugcuuucuucggaaaguaacccucgaaacaaauucagaaaugaaggaaugcaacnnnnnnnnnnnnnnnnnnnn

SEQ ID NO: 245 - RNA, 173 nt, Artificial Sequence
  sgRNA(mature form, 4bp deletion in the fourth and fifth region)
cuucacugauaaaguggagaaccgcuucaccaaaagcugucccuuaggggauuagaacuugagugaaggugggcugcuugcaucagccuaaugucgagaagugcuuucuucggaaaguaacccucgaaacaaauucgaaagaaggaaugcaacnnnnnnnnnnnnnnnnnnnn

SEQ ID NO: 246 - RNA, 171 nt, Artificial Sequence
  sgRNA(mature form, 5bp deletion in the fourth and fifth region)
cuucacugauaaaguggagaaccgcuucaccaaaagcugucccuuaggggauuagaacuugagugaaggugggcugcuugcaucagccuaaugucgagaagugcuuucuucggaaaguaacccucgaaacaaauugaaaaaggaaugcaacnnnnnnnnnnnnnnnnnnnn

SEQ ID NO: 247 - RNA, 169 nt, Artificial Sequence
  sgRNA(mature form, 6bp deletion in the fourth and fifth region)
cuucacugauaaaguggagaaccgcuucaccaaaagcugucccuuaggggauuagaacuugagugaaggugggcugcuugcaucagccuaaugucgagaagugcuuucuucggaaaguaacccucgaaacaaaugaaaaggaaugcaacnnnnnnnnnnnnnnnnnnnn

SEQ ID NO: 248 - RNA, 167 nt, Artificial Sequence
  sgRNA(mature form, 7bp deletion in the fourth and fifth region)
cuucacugauaaaguggagaaccgcuucaccaaaagcugucccuuaggggauuagaacuugagugaaggugggcugcuugcaucagccuaaugucgagaagugcuuucuucggaaaguaacccucgaaacaaagaaaggaaugcaacnnnnnnnnnnnnnnnnnnnn

SEQ ID NO: 249 - RNA, 138 nt, Artificial Sequence
  sgRNA(mature form, modified first and second region)
accgcuucaccauuagugagugaaggugggcugcuugcaucagccuaaugucgagaagugcuuucuucggaaaguaacccucgaaacaaauucauuugaaagaaugaaggaaugcaacnnnnnnnnnnnnnnnnnnnn

SEQ ID NO: 250 - RNA, 147 nt, Artificial Sequence
  sgRNA(mature form, modified first, fourth and fifth region)
accgcuucaccaaaagcugucccuuaggggauuagaacuugagugaaggugggcugcuugcaucagccuaaugucgagaagugcuuucuucggaaaguaacccucgaaacaaagaaaggaaugcaacnnnnnnnnnnnnnnnnnnnn

SEQ ID NO: 251 - RNA, 144 nt, Artificial Sequence
  sgRNA(mature form, modified second, fourth and fifth region)
cuucacugauaaaguggagaaccgcuucaccauuagugagugaaggugggcugcuugcaucagccuaaugucgagaagugcuuucuucggaaaguaacccucgaaacaaagaaaggaaugcaacnnnnnnnnnnnnnnnnnnnn

SEQ ID NO: 252 - RNA, 124 nt, Artificial Sequence
  sgRNA(mature form, modified first, second, fourth and fifth region)
accgcuucaccauuagugagugaaggugggcugcuugcaucagccuaaugucgagaagugcuuucuucggaaaguaacccucgaaacaaagaaaggaaugcaacnnnnnnnnnnnnnnnnnnnn

SEQ ID NO: 253 - RNA, 124 nt, Artificial Sequence; identical to SEQ ID NO: 252
  sgRNA(mature form, modified first, second, fourth and fifth region)

SEQ ID NO: 254 - RNA, 124 nt, Artificial Sequence; identical to SEQ ID NO: 252
  sgRNA(mature form, modified first, second, fourth and fifth region)

SEQ ID NO: 255 - RNA, 124 nt, Artificial Sequence; identical to SEQ ID NO: 252
  sgRNA(mature form, modified first, second, fourth and fifth region)

SEQ ID NO: 256 - RNA, 124 nt, Artificial Sequence; identical to SEQ ID NO: 252
  sgRNA(mature form, modified first, second, fourth and fifth region)

SEQ ID NO: 257 - RNA, 124 nt, Artificial Sequence; identical to SEQ ID NO: 252
  sgRNA(mature form, modified first, second, fourth and fifth region)

SEQ ID NO: 258 - RNA, 124 nt, Artificial Sequence; identical to SEQ ID NO: 252
  sgRNA(mature form, modified first, second, fourth and fifth region)

SEQ ID NO: 259 - protein, 529 aa, Artificial Sequence
  Cas14a1 amino acid sequence
MAKNTITKTLKLRIVRPYNSAEVEKIVADEKNNREKIALEKNKDKVKEACSKHLKVAAYCTTQVERNACLFCKARKLDDKFYQKLRGQFPDAVFWQEISEIFRQLQKQAAEIYNQSLIELYYEIFIKGKGIANASSVEHYLSDVCYTRAAELFKNAAIASGLRSKIKSNFRLKELKNMKSGLPTTKSDNFPIPLVKQKGGQYTGFEISNHNSDFIIKIPFGRWQVKKEIDKYRPWEKFDFEQVQKSPKPISLLLSTQRRKRNKGWSKDEGTEAEIKKVMNGDYQTSYIEVKRGSKIGEKSAWMLNLSIDVPKIDKGVDPSIIGGIDVGVKSPLVCAINNAFSRYSISDNDLFHFNKKMFARRRILLKKNRHKRAGHGAKNKLKPITILTEKSERFRKKLIERWACEIADFFIKNKVGTVQMENLESMKRKEDSYFNIRLRGFWPYAEMQNKIEFKLKQYGIEIRKVAPNNTSKTCSKCGHLNNYFNFEYRKKNKFPHFKCEKCNFKENADYNAALNISNPKLKSTKEEP

SEQ ID NO: 260 - protein, 536 aa, Artificial Sequence
  N-terminal NLS + Cas14a1 amino acid sequence
MPKKKRKVAKNTITKTLKLRIVRPYNSAEVEKIVADEKNNREKIALEKNKDKVKEACSKHLKVAAYCTTQVERNACLFCKARKLDDKFYQKLRGQFPDAVFWQEISEIFRQLQKQAAEIYNQSLIELYYEIFIKGKGIANASSVEHYLSDVCYTRAAELFKNAAIASGLRSKIKSNFRLKELKNMKSGLPTTKSDNFPIPLVKQKGGQYTGFEISNHNSDFIIKIPFGRWQVKKEIDKYRPWEKFDFEQVQKSPKPISLLLSTQRRKRNKGWSKDEGTEAEIKKVMNGDYQTSYIEVKRGSKIGEKSAWMLNLSIDVPKIDKGVDPSIIGGIDVGVKSPLVCAINNAFSRYSISDNDLFHFNKKMFARRRILLKKNRHKRAGHGAKNKLKPITILTEKSERFRKKLIERWACEIADFFIKNKVGTVQMENLESMKRKEDSYFNIRLRGFWPYAEMQNKIEFKLKQYGIEIRKVAPNNTSKTCSKCGHLNNYFNFEYRKKNKFPHFKCEKCNFKENADYNAALNISNPKLKSTKEEP

SEQ ID NO: 261 - protein, 536 aa, Artificial Sequence
  C-terminal NLS + Cas14a1 amino acid sequence
MAKNTITKTLKLRIVRPYNSAEVEKIVADEKNNREKIALEKNKDKVKEACSKHLKVAAYCTTQVERNACLFCKARKLDDKFYQKLRGQFPDAVFWQEISEIFRQLQKQAAEIYNQSLIELYYEIFIKGKGIANASSVEHYLSDVCYTRAAELFKNAAIASGLRSKIKSNFRLKELKNMKSGLPTTKSDNFPIPLVKQKGGQYTGFEISNHNSDFIIKIPFGRWQVKKEIDKYRPWEKFDFEQVQKSPKPISLLLSTQRRKRNKGWSKDEGTEAEIKKVMNGDYQTSYIEVKRGSKIGEKSAWMLNLSIDVPKIDKGVDPSIIGGIDVGVKSPLVCAINNAFSRYSISDNDLFHFNKKMFARRRILLKKNRHKRAGHGAKNKLKPITILTEKSERFRKKLIERWACEIADFFIKNKVGTVQMENLESMKRKEDSYFNIRLRGFWPYAEMQNKIEFKLKQYGIEIRKVAPNNTSKTCSKCGHLNNYFNFEYRKKNKFPHFKCEKCNFKENADYNAALNISNPKLKSTKEEPPKKKRKV

SEQ ID NO: 262 - protein, 543 aa, Artificial Sequence
  N/C-terminal NLS + Cas14a1 amino acid sequence
MPKKKRKVAKNTITKTLKLRIVRPYNSAEVEKIVADEKNNREKIALEKNKDKVKEACSKHLKVAAYCTTQVERNACLFCKARKLDDKFYQKLRGQFPDAVFWQEISEIFRQLQKQAAEIYNQSLIELYYEIFIKGKGIANASSVEHYLSDVCYTRAAELFKNAAIASGLRSKIKSNFRLKELKNMKSGLPTTKSDNFPIPLVKQKGGQYTGFEISNHNSDFIIKIPFGRWQVKKEIDKYRPWEKFDFEQVQKSPKPISLLLSTQRRKRNKGWSKDEGTEAEIKKVMNGDYQTSYIEVKRGSKIGEKSAWMLNLSIDVPKIDKGVDPSIIGGIDVGVKSPLVCAINNAFSRYSISDNDLFHFNKKMFARRRILLKKNRHKRAGHGAKNKLKPITILTEKSERFRKKLIERWACEIADFFIKNKVGTVQMENLESMKRKEDSYFNIRLRGFWPYAEMQNKIEFKLKQYGIEIRKVAPNNTSKTCSKCGHLNNYFNFEYRKKNKFPHFKCEKCNFKENADYNAALNISNPKLKSTKEEPPKKKRKV

SEQ ID NO: 263 - protein, 1003 aa, Artificial Sequence
  Amino acid sequence (N terminal -Cytidine deaminase)
MPKKKRKVSSETGPVAVDPTLRRRIEPHEFEVFFDPRELRKETCLLYEINWGGRHSIWRHTSQNTNKHVEVNFIEKFTTERYFCPNTRCSITWFLSWSPCGECSRAITEFLSRYPHVTLFIYIARLYHHADPRNRQGLRDLISSGVTIQIMTEQESGYCWRNFVNYSPSNEAHWPRYPHLWVRLYVLELYCIILGLPPCLNILRRKQPQLTFFTIALQSCHYQRLPPHILWATGLKSGGSSGGSSGSETPGTSESATPESSGGSSGGSAKNTITKTLKLRIVRPYNSAEVEKIVADEKNNREKIALEKNKDKVKEACSKHLKVAAYCTTQVERNACLFCKARKLDDKFYQKLRGQFPDAVFWQEISEIFRQLQKQAAEIYNQSLIELYYEIFIKGKGIANASSVEHYLSDVCYTRAAELFKNAAIASGLRSKIKSNFRLKELKNMKSGLPTTKSDNFPIPLVKQKGGQYTGFEISNHNSDFIIKIPFGRWQVKKEIDKYRPWEKFDFEQVQKSPKPISLLLSTQRRKRNKGWSKDEGTEAEIKKVMNGDYQTSYIEVKRGSKIGEKSAWMLNLSIDVPKIDKGVDPSIIGGIDVGVKSPLVCAINNAFSRYSISDNDLFHFNKKMFARRRILLKKNRHKRAGHGAKNKLKPITILTEKSERFRKKLIERWACEIADFFIKNKVGTVQMENLESMKRKEDSYFNIRLRGFWPYAEMQNKIEFKLKQYGIEIRKVAPNNTSKTCSKCGHLNNYFNFEYRKKNKFPHFKCEKCNFKENADYNAALNISNPKLKSTKEEPSGGSGGSGGSTNLSDIIEKETGKQLVIQESILMLPEEVEEVIGNKPESDILVHTAYDESTDENVMLLTSDAPEYKPWALVIQDSNGENKIKMLSGGSGGSGGSTNLSDIIEKETGKQLVIQESILMLPEEVEEVIGNKPESDILVHTAYDESTDENVMLLTSDAPEYKPWALVIQDSNGENKIKMLSGGSKRTADGSEFEPKKKRKV

SEQ ID NO: 264 - protein, 1003 aa, Artificial Sequence
  Amino acid sequence (C terminal -Cytidine deaminase)
MPKKKRKVAKNTITKTLKLRIVRPYNSAEVEKIVADEKNNREKIALEKNKDKVKEACSKHLKVAAYCTTQVERNACLFCKARKLDDKFYQKLRGQFPDAVFWQEISEIFRQLQKQAAEIYNQSLIELYYEIFIKGKGIANASSVEHYLSDVCYTRAAELFKNAAIASGLRSKIKSNFRLKELKNMKSGLPTTKSDNFPIPLVKQKGGQYTGFEISNHNSDFIIKIPFGRWQVKKEIDKYRPWEKFDFEQVQKSPKPISLLLSTQRRKRNKGWSKDEGTEAEIKKVMNGDYQTSYIEVKRGSKIGEKSAWMLNLSIDVPKIDKGVDPSIIGGIDVGVKSPLVCAINNAFSRYSISDNDLFHFNKKMFARRRILLKKNRHKRAGHGAKNKLKPITILTEKSERFRKKLIERWACEIADFFIKNKVGTVQMENLESMKRKEDSYFNIRLRGFWPYAEMQNKIEFKLKQYGIEIRKVAPNNTSKTCSKCGHLNNYFNFEYRKKNKFPHFKCEKCNFKENADYNAALNISNPKLKSTKEEPSGGSSGGSSGSETPGTSESATPESSGGSSGGSSSETGPVAVDPTLRRRIEPHEFEVFFDPRELRKETCLLYEINWGGRHSIWRHTSQNTNKHVEVNFIEKFTTERYFCPNTRCSITWFLSWSPCGECSRAITEFLSRYPHVTLFIYIARLYHHADPRNRQGLRDLISSGVTIQIMTEQESGYCWRNFVNYSPSNEAHWPRYPHLWVRLYVLELYCIILGLPPCLNILRRKQPQLTFFTIALQSCHYQRLPPHILWATGLKSGGSGGSGGSTNLSDIIEKETGKQLVIQESILMLPEEVEEVIGNKPESDILVHTAYDESTDENVMLLTSDAPEYKPWALVIQDSNGENKIKMLSGGSGGSGGSTNLSDIIEKETGKQLVIQESILMLPEEVEEVIGNKPESDILVHTAYDESTDENVMLLTSDAPEYKPWALVIQDSNGENKIKMLSGGSKRTADGSEFEPKKKRKV

SEQ ID NO: 265 - protein, 941 aa, Artificial Sequence
  DNA sequence (N terminal -Adenine deaminase)
MSEVEFSHEYWMRHALTLAKRAWDEREVPVGAVLVHNNRVIGEGWNRPIGRHDPTAHAEIMALRQGGLVMQNYRLIDATLYVTLEPCVMCAGAMIHSRIGRVVFGARDAKTGAAGSLMDVLHHPGMNHRVEITEGILADECAALLSDFFRMRRQEIKAQKKAQSSTDSGGSSGGSSGSETPGTSESATPESSGGSSGGSSEVEFSHEYWMRHALTLAKRARDEREVPVGAVLVLNNRVIGEGWNRAIGLHDPTAHAEIMALRQGGLVMQNYRLIDATLYVTFEPCVMCAGAMIHSRIGRVVFGVRNAKTGAAGSLMDVLHYPGMNHRVEITEGILADECAALLCYFFRMPRQVFNAQKKAQSSTDSGGSSGGSSGSETPGTSESATPESSGGSSGGSAKNTITKTLKLRIVRPYNSAEVEKIVADEKNNREKIALEKNKDKVKEACSKHLKVAAYCTTQVERNACLFCKARKLDDKFYQKLRGQFPDAVFWQEISEIFRQLQKQAAEIYNQSLIELYYEIFIKGKGIANASSVEHYLSDVCYTRAAELFKNAAIASGLRSKIKSNFRLKELKNMKSGLPTTKSDNFPIPLVKQKGGQYTGFEISNHNSDFIIKIPFGRWQVKKEIDKYRPWEKFDFEQVQKSPKPISLLLSTQRRKRNKGWSKDEGTEAEIKKVMNGDYQTSYIEVKRGSKIGEKSAWMLNLSIDVPKIDKGVDPSIIGGIDVGVKSPLVCAINNAFSRYSISDNDLFHFNKKMFARRRILLKKNRHKRAGHGAKNKLKPITILTEKSERFRKKLIERWACEIADFFIKNKVGTVQMENLESMKRKEDSYFNIRLRGFWPYAEMQNKIEFKLKQYGIEIRKVAPNNTSKTCSKCGHLNNYFNFEYRKKNKFPHFKCEKCNFKENADYNAALNISNPKLKSTKEEPKRPAATKKAGQAKKKK

SEQ ID NO: 266 - protein, 941 aa, Artificial Sequence
  DNA sequence (C terminal -Adenine deaminase)
MAKNTITKTLKLRIVRPYNSAEVEKIVADEKNNREKIALEKNKDKVKEACSKHLKVAAYCTTQVERNACLFCKARKLDDKFYQKLRGQFPDAVFWQEISEIFRQLQKQAAEIYNQSLIELYYEIFIKGKGIANASSVEHYLSDVCYTRAAELFKNAAIASGLRSKIKSNFRLKELKNMKSGLPTTKSDNFPIPLVKQKGGQYTGFEISNHNSDFIIKIPFGRWQVKKEIDKYRPWEKFDFEQVQKSPKPISLLLSTQRRKRNKGWSKDEGTEAEIKKVMNGDYQTSYIEVKRGSKIGEKSAWMLNLSIDVPKIDKGVDPSIIGGIDVGVKSPLVCAINNAFSRYSISDNDLFHFNKKMFARRRILLKKNRHKRAGHGAKNKLKPITILTEKSERFRKKLIERWACEIADFFIKNKVGTVQMENLESMKRKEDSYFNIRLRGFWPYAEMQNKIEFKLKQYGIEIRKVAPNNTSKTCSKCGHLNNYFNFEYRKKNKFPHFKCEKCNFKENADYNAALNISNPKLKSTKEEPSGGSSGGSSGSETPGTSESATPESSGGSSGGSSEVEFSHEYWMRHALTLAKRAWDEREVPVGAVLVHNNRVIGEGWNRPIGRHDPTAHAEIMALRQGGLVMQNYRLIDATLYVTLEPCVMCAGAMIHSRIGRVVFGARDAKTGAAGSLMDVLHHPGMNHRVEITEGILADECAALLSDFFRMRRQEIKAQKKAQSSTDSGGSSGGSSGSETPGTSESATPESSGGSSGGSSEVEFSHEYWMRHALTLAKRARDEREVPVGAVLVLNNRVIGEGWNRAIGLHDPTAHAEIMALRQGGLVMQNYRLIDATLYVTFEPCVMCAGAMIHSRIGRVVFGVRNAKTGAAGSLMDVLHYPGMNHRVEITEGILADECAALLCYFFRMPRQVFNAQKKAQSSTDKRPAATKKAGQAKKKK

SEQ ID NO: 267 - DNA, 1680 bp, Artificial Sequence
  Human codon-optimized Cas14a1 with NLS
atgccaaagaagaagcggaaggtcggtatccacggagtcccagcagccgccaagaacacaattacaaagacactgaagctgaggatcgtgagaccatacaacagcgctgaggtcgagaagattgtggctgatgaaaagaacaacagggaaaagatcgccctcgagaagaacaaggataaggtgaaggaggcctgctctaagcacctgaaagtggccgcctactgcaccacacaggtggagaggaacgcctgtctgttttgtaaagctcggaagctggatgataagttttaccagaagctgcggggccagttccccgatgccgtcttttggcaggagattagcgagatcttcagacagctgcagaagcaggccgccgagatctacaaccagagcctgatcgagctctactacgagatcttcatcaagggcaagggcattgccaacgcctcctccgtggagcactacctgagcgacgtgtgctacacaagagccgccgagctctttaagaacgccgctatcgcttccgggctgaggagcaagattaagagtaacttccggctcaaggagctgaagaacatgaagagcggcctgcccactacaaagagcgacaacttcccaattccactggtgaagcagaaggggggccagtacacagggttcgagatttccaaccacaacagcgactttattattaagatcccctttggcaggtggcaggtcaagaaggagattgacaagtacaggccctgggagaagtttgatttcgagcaggtgcagaagagccccaagcctatttccctgctgctgtccacacagcggcggaagaggaacaaggggtggtctaaggatgaggggaccgaggccgagattaagaaagtgatgaacggcgactaccagacaagctacatcgaggtcaagcggggcagtaagattggcgagaagagcgcctggatgctgaacctgagcattgacgtgccaaagattgataagggcgtggatcccagcatcatcggagggatcgatgtgggggtcaagagccccctcgtgtgcgccatcaacaacgccttcagcaggtacagcatctccgataacgacctgttccactttaacaagaagatgttcgcccggcggaggattttgctcaagaagaaccggcacaagcgggccggacacggggccaagaacaagctcaagcccatcactatcctgaccgagaagagcgagaggttcaggaagaagctcatcgagagatgggcctgcgagatcgccgatttctttattaagaacaaggtcggaacagtgcagatggagaacctcgagagcatgaagaggaaggaggattcctacttcaacattcggctgagggggttctggccctacgctgagatgcagaacaagattgagtttaagctgaagcagtacgggattgagatccggaaggtggcccccaacaacaccagcaagacctgcagcaagtgcgggcacctcaacaactacttcaacttcgagtaccggaagaagaacaagttcccacacttcaagtgcgagaagtgcaactttaaggagaacgccgattacaacgccgccctgaacatcagcaaccctaagctgaagagcactaaggaggagcccaaaaggccggcggccacgaaaaaggccggccaggcaaaaaagaaaaag

SEQ ID NO: 268 - DNA, 3009 bp, Artificial Sequence
  Deaminase fusion Cas14a1
atgccaaagaagaagcggaaagtctcctcagagactgggcctgtcgccgtcgatccaaccctgcgccgccggattgaacctcacgagtttgaagtgttctttgacccccgggagctgagaaaggagacatgcctgctgtacgagatcaactggggaggcaggcactccatctggaggcacacctctcagaacacaaataagcacgtggaggtgaacttcatcgagaagtttaccacagagcggtacttctgccccaataccagatgtagcatcacatggtttctgagctggtccccttgcggagagtgtagcagggccatcaccgagttcctgtccagatatccacacgtgacactgtttatctacatcgccaggctgtatcaccacgcagacccaaggaataggcagggcctgcgcgatctgatcagctccggcgtgaccatccagatcatgacagagcaggagtccggctactgctggcggaacttcgtgaattattctcctagcaacgaggcccactggcctaggtacccacacctgtgggtgcgcctgtacgtgctggagctgtattgcatcatcctgggcctgcccccttgtctgaatatcctgcggagaaagcagccccagctgaccttctttacaatcgccctgcagtcttgtcactatcagaggctgccaccccacatcctgtgggccacaggcctgaagtctggaggatctagcggaggatcctctggcagcgagacaccaggaacaagcgagtcagcaacaccagagagcagtggcggcagcagcggcggcagcgccaagaacacaattacaaagacactgaagctgaggatcgtgagaccatacaacagcgctgaggtcgagaagattgtggctgatgaaaagaacaacagggaaaagatcgccctcgagaagaacaaggataaggtgaaggaggcctgctctaagcacctgaaagtggccgcctactgcaccacacaggtggagaggaacgcctgtctgttttgtaaagctcggaagctggatgataagttttaccagaagctgcggggccagttccccgatgccgtcttttggcaggagattagcgagatcttcagacagctgcagaagcaggccgccgagatctacaaccagagcctgatcgagctctactacgagatcttcatcaagggcaagggcattgccaacgcctcctccgtggagcactacctgagcgacgtgtgctacacaagagccgccgagctctttaagaacgccgctatcgcttccgggctgaggagcaagattaagagtaacttccggctcaaggagctgaagaacatgaagagcggcctgcccactacaaagagcgacaacttcccaattccactggtgaagcagaaggggggccagtacacagggttcgagatttccaaccacaacagcgactttattattaagatcccctttggcaggtggcaggtcaagaaggagattgacaagtacaggccctgggagaagtttgatttcgagcaggtgcagaagagccccaagcctatttccctgctgctgtccacacagcggcggaagaggaacaaggggtggtctaaggatgaggggaccgaggccgagattaagaaagtgatgaacggcgactaccagacaagctacatcgaggtcaagcggggcagtaagattggcgagaagagcgcctggatgctgaacctgagcattgacgtgccaaagattgataagggcgtggatcccagcatcatcggagggatcgatgtgggggtcaagagccccctcgtgtgcgccatcaacaacgccttcagcaggtacagcatctccgataacgacctgttccactttaacaagaagatgttcgcccggcggaggattttgctcaagaagaaccggcacaagcgggccggacacggggccaagaacaagctcaagcccatcactatcctgaccgagaagagcgagaggttcaggaagaagctcatcgagagatgggcctgcgagatcgccgatttctttattaagaacaaggtcggaacagtgcagatggagaacctcgagagcatgaagaggaaggaggattcctacttcaacattcggctgagggggttctggccctacgctgagatgcagaacaagattgagtttaagctgaagcagtacgggattgagatccggaaggtggcccccaacaacaccagcaagacctgcagcaagtgcgggcacctcaacaactacttcaacttcgagtaccggaagaagaacaagttcccacacttcaagtgcgagaagtgcaactttaaggagaacgccgattacaacgccgccctgaacatcagcaaccctaagctgaagagcactaaggaggagcccagcggcgggagcggcgggagcggggggagcactaatctgagcgacatcattgagaaggagactgggaaacagctggtcattcaggagtccatcctgatgctgcctgaggaggtggaggaagtgatcggcaacaagccagagtctgacatcctggtgcacaccgcctacgacgagtccacagatgagaatgtgatgctgctgacctctgacgcccccgagtataagccttgggccctggtcatccaggattctaacggcgagaataagatcaagatgctgagcggaggatccggaggatctggaggcagcaccaacctgtctgacatcatcgagaaggagacaggcaagcagctggtcatccaggagagcatcctgatgctgcccgaagaagtcgaagaagtgatcggaaacaagcctgagagcgatatcctggtccataccgcctacgacgagagtaccgacgaaaatgtgatgctgctgacatccgacgccccagagtataagccctgggctctggtcatccaggattccaacggagagaacaaaatcaaaatgctgtctggcggctcaaaaagaaccgccgacggcagcgaattcgagcccaagaagaagaggaaagtc

SEQ ID NO: 269 - DNA, 1586 bp, Artificial Sequence
  human codon-optimized Cas14a1
atggccaagaacacaattacaaagacactgaagctgaggatcgtgagaccatacaacagcgctgaggtcgagaagattgtggctgatgaaaagaacaacagggaaaagatcgccctcgagaagaacaaggataaggtgaaggaggcctgctctaagcacctgaaagtggccgcctactgcaccacacaggtggagaggaacgcctgtctgttttgtaaagctcggaagctggatgataagttttaccagaagctgcggggccagttccccgatgccgtcttttggcaggagattagcgagatcttcagacagctgcagaagcaggccgccgagatctacaaccagagcctgatcgagctctactacgagatcttcatcaagggcaagggcattgccaacgcctcctccgtggagcactacctgagcgacgtgtgctacacaagagccgccgagctctttaagaacgccgctatcgcttccgggctgaggagcaagattaagagtaacttccggctcaaggagctgaagaacatgaagagcggcctgcccactacaaagagcgacaacttcccaattccactggtgaagcagaaggggggccagtacacagggttcgagatttccaaccacaacagcgactttattattaagatcccctttggcaggtggcaggtcaagaaggagattgacaagtacaggccctgggagaagtttgatttcgagcaggtgcagaagagccccaagcctatttccctgctgctgtccacacagcggcggaagaggaacaaggggtggtctaaggatgaggggaccgaggccgagattaagaaagtgatgaacggcgactaccagacaagctacatcgaggtcaagcggggcagtaagattggcgagaagagcgcctggatgctgaacctgagcattgacgtgccaaagattgataagggcgtggatcccagcatcatcggagggatcgatgtgggggtcaagagccccctcgtgtgcgccatcaacaacgccttcagcaggtacagcatctccgataacgacctgttccactttaacaagaagatgttcgcccggcggaggattttgctcaagaagaaccggcacaagcgggccggacacggggccaagaacaagctcaagcccatcactatcctgaccgagaagagcgagaggttcaggaagaagctcatcgagagatgggcctgcgagatcgccgatttctttattaagaacaaggtcggaacagtgcagatggagaacctcgagagcatgaagaggaaggaggattcctacttcaacattcggctgagggggttctggccctacgctgagatgcagaacaagattgagtttaagctgaagcagtacgggattgagatccggaaggtggcccccaacaacaccagcaagacctgcagcaagtgcgggcacctcaacaactacttcaacttcgagtaccggaagaagaacaagttcccacacttcaagtgcgagaagtgcaactttaaggagaacgccgattacaacgccgccctgaacatcagcaaccctaagctgaagagcactaaggaggagcc

SEQ ID NO: 270 - DNA, 1607 bp, Artificial Sequence
  N-terminal NLS + Cas14a1 amino acid sequence
atgccaaagaagaagcggaaagtcgccaagaacacaattacaaagacactgaagctgaggatcgtgagaccatacaacagcgctgaggtcgagaagattgtggctgatgaaaagaacaacagggaaaagatcgccctcgagaagaacaaggataaggtgaaggaggcctgctctaagcacctgaaagtggccgcctactgcaccacacaggtggagaggaacgcctgtctgttttgtaaagctcggaagctggatgataagttttaccagaagctgcggggccagttccccgatgccgtcttttggcaggagattagcgagatcttcagacagctgcagaagcaggccgccgagatctacaaccagagcctgatcgagctctactacgagatcttcatcaagggcaagggcattgccaacgcctcctccgtggagcactacctgagcgacgtgtgctacacaagagccgccgagctctttaagaacgccgctatcgcttccgggctgaggagcaagattaagagtaacttccggctcaaggagctgaagaacatgaagagcggcctgcccactacaaagagcgacaacttcccaattccactggtgaagcagaaggggggccagtacacagggttcgagatttccaaccacaacagcgactttattattaagatcccctttggcaggtggcaggtcaagaaggagattgacaagtacaggccctgggagaagtttgatttcgagcaggtgcagaagagccccaagcctatttccctgctgctgtccacacagcggcggaagaggaacaaggggtggtctaaggatgaggggaccgaggccgagattaagaaagtgatgaacggcgactaccagacaagctacatcgaggtcaagcggggcagtaagattggcgagaagagcgcctggatgctgaacctgagcattgacgtgccaaagattgataagggcgtggatcccagcatcatcggagggatcgatgtgggggtcaagagccccctcgtgtgcgccatcaacaacgccttcagcaggtacagcatctccgataacgacctgttccactttaacaagaagatgttcgcccggcggaggattttgctcaagaagaaccggcacaagcgggccggacacggggccaagaacaagctcaagcccatcactatcctgaccgagaagagcgagaggttcaggaagaagctcatcgagagatgggcctgcgagatcgccgatttctttattaagaacaaggtcggaacagtgcagatggagaacctcgagagcatgaagaggaaggaggattcctacttcaacattcggctgagggggttctggccctacgctgagatgcagaacaagattgagtttaagctgaagcagtacgggattgagatccggaaggtggcccccaacaacaccagcaagacctgcagcaagtgcgggcacctcaacaactacttcaacttcgagtaccggaagaagaacaagttcccacacttcaagtgcgagaagtgcaactttaaggagaacgccgattacaacgccgccctgaacatcagcaaccctaagctgaagagcactaaggaggagcc

SEQ ID NO: 271 - DNA, 1607 bp, Artificial Sequence
  C-terminal NLS + Cas14a1 amino acid sequence
atggccaagaacacaattacaaagacactgaagctgaggatcgtgagaccatacaacagcgctgaggtcgagaagattgtggctgatgaaaagaacaacagggaaaagatcgccctcgagaagaacaaggataaggtgaaggaggcctgctctaagcacctgaaagtggccgcctactgcaccacacaggtggagaggaacgcctgtctgttttgtaaagctcggaagctggatgataagttttaccagaagctgcggggccagttccccgatgccgtcttttggcaggagattagcgagatcttcagacagctgcagaagcaggccgccgagatctacaaccagagcctgatcgagctctactacgagatcttcatcaagggcaagggcattgccaacgcctcctccgtggagcactacctgagcgacgtgtgctacacaagagccgccgagctctttaagaacgccgctatcgcttccgggctgaggagcaagattaagagtaacttccggctcaaggagctgaagaacatgaagagcggcctgcccactacaaagagcgacaacttcccaattccactggtgaagcagaaggggggccagtacacagggttcgagatttccaaccacaacagcgactttattattaagatcccctttggcaggtggcaggtcaagaaggagattgacaagtacaggccctgggagaagtttgatttcgagcaggtgcagaagagccccaagcctatttccctgctgctgtccacacagcggcggaagaggaacaaggggtggtctaaggatgaggggaccgaggccgagattaagaaagtgatgaacggcgactaccagacaagctacatcgaggtcaagcggggcagtaagattggcgagaagagcgcctggatgctgaacctgagcattgacgtgccaaagattgataagggcgtggatcccagcatcatcggagggatcgatgtgggggtcaagagccccctcgtgtgcgccatcaacaacgccttcagcaggtacagcatctccgataacgacctgttccactttaacaagaagatgttcgcccggcggaggattttgctcaagaagaaccggcacaagcgggccggacacggggccaagaacaagctcaagcccatcactatcctgaccgagaagagcgagaggttcaggaagaagctcatcgagagatgggcctgcgagatcgccgatttctttattaagaacaaggtcggaacagtgcagatggagaacctcgagagcatgaagaggaaggaggattcctacttcaacattcggctgagggggttctggccctacgctgagatgcagaacaagattgagtttaagctgaagcagtacgggattgagatccggaaggtggcccccaacaacaccagcaagacctgcagcaagtgcgggcacctcaacaactacttcaacttcgagtaccggaagaagaacaagttcccacacttcaagtgcgagaagtgcaactttaaggagaacgccgattacaacgccgccctgaacatcagcaaccctaagctgaagagcactaaggaggagccccaaagaagaagcggaaagtc

SEQ ID NO: 272 - DNA, 1628 bp, Artificial Sequence
  N/C-terminal NLS + Cas14a1 amino acid sequence
atgccaaagaagaagcggaaagtcgccaagaacacaattacaaagacactgaagctgaggatcgtgagaccatacaacagcgctgaggtcgagaagattgtggctgatgaaaagaacaacagggaaaagatcgccctcgagaagaacaaggataaggtgaaggaggcctgctctaagcacctgaaagtggccgcctactgcaccacacaggtggagaggaacgcctgtctgttttgtaaagctcggaagctggatgataagttttaccagaagctgcggggccagttccccgatgccgtcttttggcaggagattagcgagatcttcagacagctgcagaagcaggccgccgagatctacaaccagagcctgatcgagctctactacgagatcttcatcaagggcaagggcattgccaacgcctcctccgtggagcactacctgagcgacgtgtgctacacaagagccgccgagctctttaagaacgccgctatcgcttccgggctgaggagcaagattaagagtaacttccggctcaaggagctgaagaacatgaagagcggcctgcccactacaaagagcgacaacttcccaattccactggtgaagcagaaggggggccagtacacagggttcgagatttccaaccacaacagcgactttattattaagatcccctttggcaggtggcaggtcaagaaggagattgacaagtacaggccctgggagaagtttgatttcgagcaggtgcagaagagccccaagcctatttccctgctgctgtccacacagcggcggaagaggaacaaggggtggtctaaggatgaggggaccgaggccgagattaagaaagtgatgaacggcgactaccagacaagctacatcgaggtcaagcggggcagtaagattggcgagaagagcgcctggatgctgaacctgagcattgacgtgccaaagattgataagggcgtggatcccagcatcatcggagggatcgatgtgggggtcaagagccccctcgtgtgcgccatcaacaacgccttcagcaggtacagcatctccgataacgacctgttccactttaacaagaagatgttcgcccggcggaggattttgctcaagaagaaccggcacaagcgggccggacacggggccaagaacaagctcaagcccatcactatcctgaccgagaagagcgagaggttcaggaagaagctcatcgagagatgggcctgcgagatcgccgatttctttattaagaacaaggtcggaacagtgcagatggagaacctcgagagcatgaagaggaaggaggattcctacttcaacattcggctgagggggttctggccctacgctgagatgcagaacaagattgagtttaagctgaagcagtacgggattgagatccggaaggtggcccccaacaacaccagcaagacctgcagcaagtgcgggcacctcaacaactacttcaacttcgagtaccggaagaagaacaagttcccacacttcaagtgcgagaagtgcaactttaaggagaacgccgattacaacgccgccctgaacatcagcaaccctaagctgaagagcactaaggaggagccccaaagaagaagcggaaagtc

SEQ ID NO: 273 - DNA, 3009 bp, Artificial Sequence; identical to SEQ ID NO: 268
  Amino acid sequence (N terminal -Cytidine deaminase)

SEQ ID NO: 274 - DNA, 3009 bp, Artificial Sequence
  Amino acid sequence (C terminal -Cytidine deaminase)
atgccaaagaagaagcggaaagtcgccaagaacacaattacaaagacactgaagctgaggatcgtgagaccatacaacagcgctgaggtcgagaagattgtggctgatgaaaagaacaacagggaaaagatcgccctcgagaagaacaaggataaggtgaaggaggcctgctctaagcacctgaaagtggccgcctactgcaccacacaggtggagaggaacgcctgtctgttttgtaaagctcggaagctggatgataagttttaccagaagctgcggggccagttccccgatgccgtcttttggcaggagattagcgagatcttcagacagctgcagaagcaggccgccgagatctacaaccagagcctgatcgagctctactacgagatcttcatcaagggcaagggcattgccaacgcctcctccgtggagcactacctgagcgacgtgtgctacacaagagccgccgagctctttaagaacgccgctatcgcttccgggctgaggagcaagattaagagtaacttccggctcaaggagctgaagaacatgaagagcggcctgcccactacaaagagcgacaacttcccaattccactggtgaagcagaaggggggccagtacacagggttcgagatttccaaccacaacagcgactttattattaagatcccctttggcaggtggcaggtcaagaaggagattgacaagtacaggccctgggagaagtttgatttcgagcaggtgcagaagagccccaagcctatttccctgctgctgtccacacagcggcggaagaggaacaaggggtggtctaaggatgaggggaccgaggccgagattaagaaagtgatgaacggcgactaccagacaagctacatcgaggtcaagcggggcagtaagattggcgagaagagcgcctggatgctgaacctgagcattgacgtgccaaagattgataagggcgtggatcccagcatcatcggagggatcgatgtgggggtcaagagccccctcgtgtgcgccatcaacaacgccttcagcaggtacagcatctccgataacgacctgttccactttaacaagaagatgttcgcccggcggaggattttgctcaagaagaaccggcacaagcgggccggacacggggccaagaacaagctcaagcccatcactatcctgaccgagaagagcgagaggttcaggaagaagctcatcgagagatgggcctgcgagatcgccgatttctttattaagaacaaggtcggaacagtgcagatggagaacctcgagagcatgaagaggaaggaggattcctacttcaacattcggctgagggggttctggccctacgctgagatgcagaacaagattgagtttaagctgaagcagtacgggattgagatccggaaggtggcccccaacaacaccagcaagacctgcagcaagtgcgggcacctcaacaactacttcaacttcgagtaccggaagaagaacaagttcccacacttcaagtgcgagaagtgcaactttaaggagaacgccgattacaacgccgccctgaacatcagcaaccctaagctgaagagcactaaggaggagccctctggaggatctagcggaggatcctctggcagcgagacaccaggaacaagcgagtcagcaacaccagagagcagtggcggcagcagcggcggcagctcctcagagactgggcctgtcgccgtcgatccaaccctgcgccgccggattgaacctcacgagtttgaagtgttctttgacccccgggagctgagaaaggagacatgcctgctgtacgagatcaactggggaggcaggcactccatctggaggcacacctctcagaacacaaataagcacgtggaggtgaacttcatcgagaagtttaccacagagcggtacttctgccccaataccagatgtagcatcacatggtttctgagctggtccccttgcggagagtgtagcagggccatcaccgagttcctgtccagatatccacacgtgacactgtttatctacatcgccaggctgtatcaccacgcagacccaaggaataggcagggcctgcgcgatctgatcagctccggcgtgaccatccagatcatgacagagcaggagtccggctactgctggcggaacttcgtgaattattctcctagcaacgaggcccactggcctaggtacccacacctgtgggtgcgcctgtacgtgctggagctgtattgcatcatcctgggcctgcccccttgtctgaatatcctgcggagaaagcagccccagctgaccttctttacaatcgccctgcagtcttgtcactatcagaggctgccaccccacatcctgtgggccacaggcctgaagagcggcgggagcggcgggagcggggggagcactaatctgagcgacatcattgagaaggagactgggaaacagctggtcattcaggagtccatcctgatgctgcctgaggaggtggaggaagtgatcggcaacaagccagagtctgacatcctggtgcacaccgcctacgacgagtccacagatgagaatgtgatgctgctgacctctgacgcccccgagtataagccttgggccctggtcatccaggattctaacggcgagaataagatcaagatgctgagcggaggatccggaggatctggaggcagcaccaacctgtctgacatcatcgagaaggagacaggcaagcagctggtcatccaggagagcatcctgatgctgcccgaagaagtcgaagaagtgatcggaaacaagcctgagagcgatatcctggtccataccgcctacgacgagagtaccgacgaaaatgtgatgctgctgacatccgacgccccagagtataagccctgggctctggtcatccaggattccaacggagagaacaaaatcaaaatgctgtctggcggctcaaaaagaaccgccgacggcagcgaattcgagcccaagaagaagaggaaagtc

SEQ ID NO: 275 - DNA, 2823 bp, Artificial Sequence
  DNA sequence (N terminal -Adenine deaminase)
atgtccgaagtcgagttttcccatgagtactggatgagacacgcattgactctcgcaaagagggcttgggatgaacgcgaggtgcccgtgggggcagtactcgtgcataacaatcgcgtaatcggcgaaggttggaataggccgatcggacgccacgaccccactgcacatgcggaaatcatggcccttcgacagggagggcttgtgatgcagaattatcgacttatcgatgcgacgctgtacgtcacgcttgaaccttgcgtaatgtgcgcgggagctatgattcactcccgcattggacgagttgtattcggtgcccgcgacgccaagacgggtgccgcaggttcactgatggacgtgctgcatcacccaggcatgaaccaccgggtagaaatcacagaaggcatattggcggacgaatgtgcggcgctgttgtccgacttttttcgcatgcggaggcaggagatcaaggcccagaaaaaagcacaatcctctactgactctggtggttcttctggtggttctagcggcagcgagactcccgggacctcagagtccgccacacccgaaagttctggtggttcttctggtggttcttccgaagtcgagttttcccatgagtactggatgagacacgcattgactctcgcaaagagggctcgagatgaacgcgaggtgcccgtgggggcagtactcgtgctcaacaatcgcgtaatcggcgaaggttggaatagggcaatcggactccacgaccccactgcacatgcggaaatcatggcccttcgacagggagggcttgtgatgcagaattatcgacttatcgatgcgacgctgtacgtcacgtttgaaccttgcgtaatgtgcgcgggagctatgattcactcccgcattggacgagttgtattcggtgttcgcaacgccaagacgggtgccgcaggttcactgatggacgtgctgcattacccaggcatgaaccaccgggtagaaatcacagaaggcatattggcggacgaatgtgcggcgctgttgtgttacttttttcgcatgcccaggcaggtctttaacgcccagaaaaaagcacaatcctctactgactctggtggttcttctggtggttctagcggcagcgagactcccgggacctcagagtccgccacacccgaaagttctggtggttcttctggtggttctgccaagaacacaattacaaagacactgaagctgaggatcgtgagaccatacaacagcgctgaggtcgagaagattgtggctgatgaaaagaacaacagggaaaagatcgccctcgagaagaacaaggataaggtgaaggaggcctgctctaagcacctgaaagtggccgcctactgcaccacacaggtggagaggaacgcctgtctgttttgtaaagctcggaagctggatgataagttttaccagaagctgcggggccagttccccgatgccgtcttttggcaggagattagcgagatcttcagacagctgcagaagcaggccgccgagatctacaaccagagcctgatcgagctctactacgagatcttcatcaagggcaagggcattgccaacgcctcctccgtggagcactacctgagcgacgtgtgctacacaagagccgccgagctctttaagaacgccgctatcgcttccgggctgaggagcaagattaagagtaacttccggctcaaggagctgaagaacatgaagagcggcctgcccactacaaagagcgacaacttcccaattccactggtgaagcagaaggggggccagtacacagggttcgagatttccaaccacaacagcgactttattattaagatcccctttggcaggtggcaggtcaagaaggagattgacaagtacaggccctgggagaagtttgatttcgagcaggtgcagaagagccccaagcctatttccctgctgctgtccacacagcggcggaagaggaacaaggggtggtctaaggatgaggggaccgaggccgagattaagaaagtgatgaacggcgactaccagacaagctacatcgaggtcaagcggggcagtaagattggcgagaagagcgcctggatgctgaacctgagcattgacgtgccaaagattgataagggcgtggatcccagcatcatcggagggatcgatgtgggggtcaagagccccctcgtgtgcgccatcaacaacgccttcagcaggtacagcatctccgataacgacctgttccactttaacaagaagatgttcgcccggcggaggattttgctcaagaagaaccggcacaagcgggccggacacggggccaagaacaagctcaagcccatcactatcctgaccgagaagagcgagaggttcaggaagaagctcatcgagagatgggcctgcgagatcgccgatttctttattaagaacaaggtcggaacagtgcagatggagaacctcgagagcatgaagaggaaggaggattcctacttcaacattcggctgagggggttctggccctacgctgagatgcagaacaagattgagtttaagctgaagcagtacgggattgagatccggaaggtggcccccaacaacaccagcaagacctgcagcaagtgcgggcacctcaacaactacttcaacttcgagtaccggaagaagaacaagttcccacacttcaagtgcgagaagtgcaactttaaggagaacgccgattacaacgccgccctgaacatcagcaaccctaagctgaagagcactaaggaggagcccaaaaggccggcggccacgaaaaaggccggccaggcaaaaaagaaaaag

SEQ ID NO: 276 - DNA, 2823 bp, Artificial Sequence
  DNA sequence (C terminal -Adenine deaminase)
atggccaagaacacaattacaaagacactgaagctgaggatcgtgagaccatacaacagcgctgaggtcgagaagattgtggctgatgaaaagaacaacagggaaaagatcgccctcgagaagaacaaggataaggtgaaggaggcctgctctaagcacctgaaagtggccgcctactgcaccacacaggtggagaggaacgcctgtctgttttgtaaagctcggaagctggatgataagttttaccagaagctgcggggccagttccccgatgccgtcttttggcaggagattagcgagatcttcagacagctgcagaagcaggccgccgagatctacaaccagagcctgatcgagctctactacgagatcttcatcaagggcaagggcattgccaacgcctcctccgtggagcactacctgagcgacgtgtgctacacaagagccgccgagctctttaagaacgccgctatcgcttccgggctgaggagcaagattaagagtaacttccggctcaaggagctgaagaacatgaagagcggcctgcccactacaaagagcgacaacttcccaattccactggtgaagcagaaggggggccagtacacagggttcgagatttccaaccacaacagcgactttattattaagatcccctttggcaggtggcaggtcaagaaggagattgacaagtacaggccctgggagaagtttgatttcgagcaggtgcagaagagccccaagcctatttccctgctgctgtccacacagcggcggaagaggaacaaggggtggtctaaggatgaggggaccgaggccgagattaagaaagtgatgaacggcgactaccagacaagctacatcgaggtcaagcggggcagtaagattggcgagaagagcgcctggatgctgaacctgagcattgacgtgccaaagattgataagggcgtggatcccagcatcatcggagggatcgatgtgggggtcaagagccccctcgtgtgcgccatcaacaacgccttcagcaggtacagcatctccgataacgacctgttccactttaacaagaagatgttcgcccggcggaggattttgctcaagaagaaccggcacaagcgggccggacacggggccaagaacaagctcaagcccatcactatcctgaccgagaagagcgagaggttcaggaagaagctcatcgagagatgggcctgcgagatcgccgatttctttattaagaacaaggtcggaacagtgcagatggagaacctcgagagcatgaagaggaaggaggattcctacttcaacattcggctgagggggttctggccctacgctgagatgcagaacaagattgagtttaagctgaagcagtacgggattgagatccggaaggtggcccccaacaacaccagcaagacctgcagcaagtgcgggcacctcaacaactacttcaacttcgagtaccggaagaagaacaagttcccacacttcaagtgcgagaagtgcaactttaaggagaacgccgattacaacgccgccctgaacatcagcaaccctaagctgaagagcactaaggaggagccctctggaggatctagcggaggatcctctggcagcgagacaccaggaacaagcgagtcagcaacaccagagagcagtggcggcagcagcggcggcagctccgaagtcgagttttcccatgagtactggatgagacacgcattgactctcgcaaagagggcttgggatgaacgcgaggtgcccgtgggggcagtactcgtgcataacaatcgcgtaatcggcgaaggttggaataggccgatcggacgccacgaccccactgcacatgcggaaatcatggcccttcgacagggagggcttgtgatgcagaattatcgacttatcgatgcgacgctgtacgtcacgcttgaaccttgcgtaatgtgcgcgggagctatgattcactcccgcattggacgagttgtattcggtgcccgcgacgccaagacgggtgccgcaggttcactgatggacgtgctgcatcacccaggcatgaaccaccgggtagaaatcacagaaggcatattggcggacgaatgtgcggcgctgttgtccgacttttttcgcatgcggaggcaggagatcaaggcccagaaaaaagcacaatcctctactgactctggtggttcttctggtggttctagcggcagcgagactcccgggacctcagagtccgccacacccgaaagttcaggtggatcttcaggtggatcttcggaagtggaattttcgcacgagtattggatgaggcacgctttaactctcgctaagagagcacgagacgaacgggaagtgccggttggggctgtcctcgtactcaataatcgagttatcggagaaggctggaacagggcaatcggactccacgatcccacagctcatgccgagataatggcgcttcgacaaggaggcctagtcatgcaaaattatcgtcttattgacgcgaccctctacgtgacctttgagccatgcgttatgtgtgcgggtgcaatgatacattcccggataggacgtgtagtatttggagttcgcaacgcgaagaccggtgcggctggttctctcatggatgtcctgcactaccctgggatgaatcaccgcgttgaaatcactgaaggcattttggccgatgaatgcgcggccctgttatgttacttttttcgcatgcccaggcaggtctttaacgcacagaagaaagcccaatcgtccactgataaaaggccggcggccacgaaaaaggccggccaggcaaaaaagaaaaag

SEQ ID NO: 277 - protein, 7 aa, simian virus 40
PKKKRKV

SEQ ID NO: 278 - protein, 16 aa, mus musculus
KRPAATKKAGQAKKKK

SEQ ID NO: 279 - protein, 9 aa, homo sapiens
PAAKRVKLD

SEQ ID NO: 280 - protein, 11 aa, homo sapiens
RQRRNELKRSP

SEQ ID NO: 281 - protein, 38 aa, mus musculus
NQSSNFGPMKGGNFGGRSSGPYGGGGQYFAKPRNQGGY

SEQ ID NO: 282 - protein, 42 aa, Homo sapiens
RMRIZFKNKGKDTAELRRRRVEVSVELRKAKKDEQILKRRNV

SEQ ID NO: 283 - protein, 8 aa, Homo sapiens
VSRKRPRP

SEQ ID NO: 284 - protein, 8 aa, homo sapiens
PPKKARED

SEQ ID NO: 285 - protein, 8 aa, homo sapiens
PQPKKKPL

SEQ ID NO: 286 - protein, 12 aa, mus musculus
SALIKKKKKMAP

SEQ ID NO: 287 - protein, 5 aa, Influenza virus
DRLRR

SEQ ID NO: 288 - protein, 7 aa, influenza virus
PKQKKRK

SEQ ID NO: 289 - protein, 10 aa, Hepatitis D virus
RKLKKKIKKL

SEQ ID NO: 290 - protein, 10 aa, mus musculus
REKKKFLKRR

SEQ ID NO: 291 - protein, 20 aa, homo sapiens
KRKGDEVDGVDEVAKKKSKK

SEQ ID NO: 292 - protein, 17 aa, Homo sapiens
RKCLQAGMNLEARKTKK

SEQ ID NO: 293 - RNA, 29 nt, Artificial Sequence
  engineered (4th region + Linker + 5th region) of WT gRNA
aacaaauucauuuugaaacgaaugaagga

SEQ ID NO: 294 - RNA, 31 nt, Artificial Sequence
  engineered (4th region + Linker + 5th region) of WT gRNA
aacaaauucauuuuugaaaacgaaugaagga

SEQ ID NO: 295 - RNA, 33 nt, Artificial Sequence
  engineered (4th region + Linker + 5th region) of WT gRNA
aacaaauucauuuuucgaaagacgaaugaagga

SEQ ID NO: 296 - RNA, 35 nt, Artificial Sequence
  engineered (4th region + Linker + 5th region) of WT gRNA
aacaaauucauuuuuccgaaaagacgaaugaagga

SEQ ID NO: 297 - RNA, 37 nt, Artificial Sequence
  engineered (4th region + Linker + 5th region) of WT gRNA
aacaaauucauuuuuccugaaauagacgaaugaagga

SEQ ID NO: 298 - RNA, 39 nt, Artificial Sequence
  engineered (4th region + Linker + 5th region) of WT gRNA
aacaaauucauuuuuccucgaaaauagacgaaugaagga

SEQ ID NO: 299 - RNA, 41 nt, Artificial Sequence
  engineered (4th region + Linker + 5th region) of WT gRNA
aacaaauucauuuuuccucugaaaaauagacgaaugaagga

SEQ ID NO: 300 - RNA, 43 nt, Artificial Sequence
  engineered (4th region + Linker + 5th region) of WT gRNA
aacaaauucauuuuuccucucgaaagaauagacgaaugaagga

SEQ ID NO: 301 - RNA, 45 nt, Artificial Sequence
  engineered (4th region + Linker + 5th region) of WT gRNA
aacaaauucauuuuuccucuccgaaacgaauagacgaaugaagga

SEQ ID NO: 302 - RNA, 47 nt, Artificial Sequence
  engineered (4th region + Linker + 5th region) of WT gRNA
aacaaauucauuuuuccucuccagaaaccgaauagacgaaugaagga

SEQ ID NO: 303 - RNA, 49 nt, Artificial Sequence
  engineered (4th region + Linker + 5th region) of WT gRNA
aacaaauucauuuuuccucuccaagaaacccgaauagacgaaugaagga

SEQ ID NO: 304 - RNA, 51 nt, Artificial Sequence
  engineered (4th region + Linker + 5th region) of WT gRNA
aacaaauucauuuuuccucuccaaugaaaacccgaauagacgaaugaagga

SEQ ID NO: 305 - RNA, 53 nt, Artificial Sequence
  engineered (4th region + Linker + 5th region) of WT gRNA
aacaaauucauuuuuccucuccaauugaaaaacccgaauagacgaaugaagga

SEQ ID NO: 306 - RNA, 55 nt, Artificial Sequence
  engineered (4th region + Linker + 5th region) of WT gRNA
aacaaauucauuuuuccucuccaauucgaaagaacccgaauagacgaaugaagga

SEQ ID NO: 307 - RNA, 57 nt, Artificial Sequence
  engineered (4th region + Linker + 5th region) of WT gRNA
aacaaauucauuuuuccucuccaauucugaaaagaacccgaauagacgaaugaagga

SEQ ID NO: 308 - RNA, 59 nt, Artificial Sequence
  engineered (4th region + Linker + 5th region) of WT gRNA
aacaaauucauuuuuccucuccaauucuggaaacagaacccgaauagacgaaugaagga

SEQ ID NO: 309 - RNA, 61 nt, Artificial Sequence
  engineered (4th region + Linker + 5th region) of WT gRNA
aacaaauucauuuuuccucuccaauucugcgaaagcagaacccgaauagacgaaugaagga

SEQ ID NO: 310 - RNA, 63 nt, Artificial Sequence
  engineered (4th region + Linker + 5th region) of WT gRNA
aacaaauucauuuuuccucuccaauucugcagaaaugcagaacccgaauagacgaaugaagga

SEQ ID NO: 311 - RNA, 65 nt, Artificial Sequence
  engineered (4th region + Linker + 5th region) of WT gRNA
aacaaauucauuuuuccucuccaauucugcacgaaauugcagaacccgaauagacgaaugaagga

SEQ ID NO: 312 - RNA, 67 nt, Artificial Sequence
  engineered (4th region + Linker + 5th region) of WT gRNA
aacaaauucauuuuuccucuccaauucugcacagaaaguugcagaacccgaauagacgaaugaagga

SEQ ID NO: 313 - RNA, 66 nt, Artificial Sequence
  engineered (4th region + Linker + 5th region) of WT gRNA
aacaaauucauuuuuccucuccaauucugcacagaaauugcagaacccgaauagacgaaugaagga

SEQ ID NO: 314 - RNA, 68 nt, Artificial Sequence
  (4th region + Linker + 5th region) of WT gRNA
aacaaauucauuuuuccucuccaauucugcacaagaaaguugcagaacccgaauagacgaaugaagga

SEQ ID NO: 315 - RNA, 202 nt, Artificial Sequence
  wild-type of Cas12f1 tracrRNA + GAAA + wild-type of Cas12f1 crRNA repeat
cuucacugauaaaguggagaaccgcuucaccaaaagcugucccuuaggggauuagaacuugagugaaggugggcugcuugcaucagccuaaugucgagaagugcuuucuucggaaaguaacccucgaaacaaauucauuuuuccucuccaauucugcacaagaaaguugcagaacccgaauagacgaaugaaggaaugcaac

SEQ ID NO: 316 - RNA, 10 nt, Artificial Sequence
  Linker variation, WT
caagaaaguu

SEQ ID NO: 317 - RNA, 12 nt, Artificial Sequence
  Linker variation, WT
acaagaaaguug

SEQ ID NO: 318 - RNA, 14 nt, Artificial Sequence
  Linker variation, WT
cacaagaaaguugc

SEQ ID NO: 319 - RNA, 16 nt, Artificial Sequence
  Linker variation, WT
gcacaagaaaguugca

SEQ ID NO: 320 - RNA, 18 nt, Artificial Sequence
  Linker variation, WT
ugcacaagaaaguugcag

SEQ ID NO: 321 - RNA, 20 nt, Artificial Sequence
  Linker variation, WT
cugcacaagaaaguugcaga

SEQ ID NO: 322 - RNA, 22 nt, Artificial Sequence
  Linker variation, WT
ucugcacaagaaaguugcagaa

SEQ ID NO: 323 - RNA, 24 nt, Artificial Sequence
  Linker variation, WT
uucugcacaagaaaguugcagaac

SEQ ID NO: 324 - RNA, 26 nt, Artificial Sequence
  Linker variation, WT
auucugcacaagaaaguugcagaacc

SEQ ID NO: 325 - RNA, 28 nt, Artificial Sequence
  Linker variation, WT
aauucugcacaagaaaguugcagaaccc

SEQ ID NO: 326 - RNA, 30 nt, Artificial Sequence
  Linker variation, WT
caauucugcacaagaaaguugcagaacccg

SEQ ID NO: 327 - RNA, 32 nt, Artificial Sequence
  Linker variation, WT
ccaauucugcacaagaaaguugcagaacccga

SEQ ID NO: 328 - RNA, 34 nt, Artificial Sequence
  Linker variation, WT
uccaauucugcacaagaaaguugcagaacccgaa

SEQ ID NO: 329 - RNA, 36 nt, Artificial Sequence
  Linker variation, WT
cuccaauucugcacaagaaaguugcagaacccgaau

SEQ ID NO: 330 - RNA, 38 nt, Artificial Sequence
  Linker variation, WT
ucuccaauucugcacaagaaaguugcagaacccgaaua

SEQ ID NO: 331 - RNA, 40 nt, Artificial Sequence
  Linker variation, WT
cucuccaauucugcacaagaaaguugcagaacccgaauag

SEQ ID NO: 332 - RNA, 42 nt, Artificial Sequence
  Linker variation, WT
ccucuccaauucugcacaagaaaguugcagaacccgaauaga

SEQ ID NO: 333 - RNA, 44 nt, Artificial Sequence
  Linker variation, WT
uccucuccaauucugcacaagaaaguugcagaacccgaauagac

SEQ ID NO: 334 - RNA, 46 nt, Artificial Sequence
  Linker variation, WT
uuccucuccaauucugcacaagaaaguugcagaacccgaauagacg

SEQ ID NO: 335 - RNA, 48 nt, Artificial Sequence
  Linker variation, WT
uuuccucuccaauucugcacaagaaaguugcagaacccgaauagacga

SEQ ID NO: 336 - RNA, 50 nt, Artificial Sequence
  Linker variation, WT
uuuuccucuccaauucugcacaagaaaguugcagaacccgaauagacgaa

SEQ ID NO: 337 - RNA, 52 nt, Artificial Sequence
  Linker variation, WT
uuuuuccucuccaauucugcacaagaaaguugcagaacccgaauagacgaau

SEQ ID NO: 338 - RNA, 54 nt, Artificial Sequence
  Linker variation, WT
auuuuuccucuccaauucugcacaagaaaguugcagaacccgaauagacgaaug

SEQ ID NO: 339 - RNA, 56 nt, Artificial Sequence
  Linker variation, WT
cauuuuuccucuccaauucugcacaagaaaguugcagaacccgaauagacgaauga

SEQ ID NO: 340 - RNA, 58 nt, Artificial Sequence
  Linker variation, WT
ucauuuuuccucuccaauucugcacaagaaaguugcagaacccgaauagacgaaugaa

SEQ ID NO: 341 - RNA, 57 nt, Artificial Sequence
  Linker variation, WT
ucauuuuuccucuccaauucugcacaagaaaguugcagaacccgaauagacgaauga

SEQ ID NO: 342 - RNA, 59 nt, Artificial Sequence
  Linker variation, WT
uucauuuuuccucuccaauucugcacaagaaaguugcagaacccgaauagacgaaugaa

SEQ ID NO: 343 - RNA, 10 nt, Artificial Sequence
  deleted part of 4th region, WT
uucauuuuuc

SEQ ID NO: 344 - RNA, 11 nt, Artificial Sequence
  deleted part of 4th region, WT
uucauuuuucc

SEQ ID NO: 345 - RNA, 12 nt, Artificial Sequence
  deleted part of 4th region, WT
uucauuuuuccu

SEQ ID NO: 346 - RNA, 13 nt, Artificial Sequence
  deleted part of 4th region, WT
uucauuuuuccuc

SEQ ID NO: 347 - RNA, 14 nt, Artificial Sequence
  deleted part of 4th region, WT
uucauuuuuccucu

SEQ ID NO: 348 - RNA, 15 nt, Artificial Sequence
  deleted part of 4th region, WT
uucauuuuuccucuc

SEQ ID NO: 349 - RNA, 16 nt, Artificial Sequence
  deleted part of 4th region, WT
uucauuuuuccucucc

SEQ ID NO: 350 - RNA, 17 nt, Artificial Sequence
  deleted part of 4th region, WT
uucauuuuuccucucca

SEQ ID NO: 351 - RNA, 18 nt, Artificial Sequence
  deleted part of 4th region, WT
uucauuuuuccucuccaa

SEQ ID NO: 352 - RNA, 19 nt, Artificial Sequence
  deleted part of 4th region, WT
uucauuuuuccucuccaau

SEQ ID NO: 353 - RNA, 20 nt, Artificial Sequence
  deleted part of 4th region, WT
uucauuuuuccucuccaauu

SEQ ID NO: 354 - RNA, 21 nt, Artificial Sequence
  deleted part of 4th region, WT
uucauuuuuccucuccaauuc

SEQ ID NO: 355 - RNA, 22 nt, Artificial Sequence
  deleted part of 4th region, WT
uucauuuuuccucuccaauucu

SEQ ID NO: 356 - RNA, 23 nt, Artificial Sequence
  deleted part of 4th region, WT
uucauuuuuccucuccaauucug

SEQ ID NO: 357 - RNA, 24 nt, Artificial Sequence
  deleted part of 4th region, WT
uucauuuuuccucuccaauucugc

SEQ ID NO: 358 - RNA, 25 nt, Artificial Sequence
  deleted part of 4th region, WT
uucauuuuuccucuccaauucugca

SEQ ID NO: 359 - RNA, 26 nt, Artificial Sequence
  deleted part of 4th region, WT
uucauuuuuccucuccaauucugcac

SEQ ID NO: 360 - RNA, 27 nt, Artificial Sequence
  deleted part of 4th region, WT
uucauuuuuccucuccaauucugcaca

SEQ ID NO: 361 - RNA, 28 nt, Artificial Sequence
  deleted part of 4th region, WT
uucauuuuuccucuccaauucugcacaa

SEQ ID NO: 362 - RNA, 10 nt, Artificial Sequence
  deleted part of 5th region, WT
gacgaaugaa

SEQ ID NO: 363 - RNA, 11 nt, Artificial Sequence
  deleted part of 5th region, WT
agacgaaugaa

SEQ ID NO: 364 - RNA, 12 nt, Artificial Sequence
  deleted part of 5th region, WT
uagacgaaugaa

SEQ ID NO: 365 - RNA, 13 nt, Artificial Sequence
  deleted part of 5th region, WT
auagacgaaugaa

SEQ ID NO: 366 - RNA, 14 nt, Artificial Sequence
  deleted part of 5th region, WT
aauagacgaaugaa

SEQ ID NO: 367 - RNA, 15 nt, Artificial Sequence
  deleted part of 5th region, WT
gaauagacgaaugaa

SEQ ID NO: 368 - RNA, 16 nt, Artificial Sequence
  deleted part of 5th region, WT
cgaauagacgaaugaa

SEQ ID NO: 369 - RNA, 17 nt, Artificial Sequence
  deleted part of 5th region, WT
ccgaauagacgaaugaa

SEQ ID NO: 370 - RNA, 18 nt, Artificial Sequence
  deleted part of 5th region, WT
cccgaauagacgaaugaa

SEQ ID NO: 371 - RNA, 19 nt, Artificial Sequence
  deleted part of 5th region, WT
acccgaauagacgaaugaa

SEQ ID NO: 372 - RNA, 20 nt, Artificial Sequence
  deleted part of 5th region, WT
aacccgaauagacgaaugaa

SEQ ID NO: 373 - RNA, 21 nt, Artificial Sequence
  deleted part of 5th region, WT
gaacccgaauagacgaaugaa

SEQ ID NO: 374 - RNA, 22 nt, Artificial Sequence
  deleted part of 5th region, WT
agaacccgaauagacgaaugaa

SEQ ID NO: 375 - RNA, 23 nt, Artificial Sequence
  deleted part of 5th region, WT
cagaacccgaauagacgaaugaa

SEQ ID NO: 376 - RNA, 24 nt, Artificial Sequence
  deleted part of 5th region, WT
gcagaacccgaauagacgaaugaa

SEQ ID NO: 377 - RNA, 25 nt, Artificial Sequence
  deleted part of 5th region, WT
ugcagaacccgaauagacgaaugaa

SEQ ID NO: 378 - RNA, 26 nt, Artificial Sequence
  deleted part of 5th region, WT
uugcagaacccgaauagacgaaugaa

SEQ ID NO: 379 - RNA, 27 nt, Artificial Sequence
  deleted part of 5th region, WT
guugcagaacccgaauagacgaaugaa

SEQ ID NO: 380 - RNA, 181 nt, Artificial Sequence
  Comparative Example 1.1
cuucacugauaaaguggagaaccgcuucaccaaaagcugucccuuaggggauuagaacuugagugaaggugggcugcuugcaucagccuaaugucgagaagugcuuucuucggaaaguaacccucgaaacaaauucauuugaaagaaugaaggaaugcaaccacacacacagugggcuacc

SEQ ID NO: 381 - RNA, 174 nt, Artificial Sequence
  Example 1.1
gauaaaguggagaaccgcuucaccaaaagcugucccuuaggggauuagaacuugagugaaggugggcugcuugcaucagccuaaugucgagaagugcuuucuucggaaaguaacccucgaaacaaauucauuugaaagaaugaaggaaugcaaccacacacacagugggcuacc

SEQ ID NO: 382 - RNA, 167 nt, Artificial Sequence
  Example 1.2
uggagaaccgcuucaccaaaagcugucccuuaggggauuagaacuugagugaaggugggcugcuugcaucagccuaaugucgagaagugcuuucuucggaaaguaacccucgaaacaaauucauuugaaagaaugaaggaaugcaaccacacacacagugggcuacc

SEQ ID NO: 383 - RNA, 161 nt, Artificial Sequence
  Example 1.3
accgcuucaccaaaagcugucccuuaggggauuagaacuugagugaaggugggcugcuugcaucagccuaaugucgagaagugcuuucuucggaaaguaacccucgaaacaaauucauuugaaagaaugaaggaaugcaaccacacacacagugggcuacc

SEQ ID NO: 384 - RNA, 175 nt, Artificial Sequence
  Example 1.4
cuucacugauaaaguggagaaccgcuucaccaaaagcuguuuagauuagaacuugagugaaggugggcugcuugcaucagccuaaugucgagaagugcuuucuucggaaaguaacccucgaaacaaauucauuugaaagaaugaaggaaugcaaccacacacacagugggcuacc

SEQ ID NO: 385 - RNA, 170 nt, Artificial Sequence
  Example 1.5
cuucacugauaaaguggagaaccgcuucaccaaaagcuuuagagaacuugagugaaggugggcugcuugcaucagccuaaugucgagaagugcuuucuucggaaaguaacccucgaaacaaauucauuugaaagaaugaaggaaugcaaccacacacacagugggcuacc

SEQ ID NO: 386 - RNA, 158 nt, Artificial Sequence
  Example 1.6
cuucacugauaaaguggagaaccgcuucaccauuagugagugaaggugggcugcuugcaucagccuaaugucgagaagugcuuucuucggaaaguaacccucgaaacaaauucauuugaaagaaugaaggaaugcaaccacacacacagugggcuacc

SEQ ID NO: 387 - RNA, 177 nt, Artificial Sequence
  Example 1.7
cuucacugauaaaguggagaaccgcuucaccaaaagcugucccuuaggggauuagaacuugagugaaggugggcugcuugcaucagccuaaugucgagaagugcuuucuucggaaaguaacccucgaaacaaauucaugaaaaugaaggaaugcaaccacacacacagugggcuacc

SEQ ID NO: 388 - RNA, 173 nt, Artificial Sequence
  Example 1.8
cuucacugauaaaguggagaaccgcuucaccaaaagcugucccuuaggggauuagaacuugagugaaggugggcugcuugcaucagccuaaugucgagaagugcuuucuucggaaaguaacccucgaaacaaauucgaaagaaggaaugcaaccacacacacagugggcuacc

SEQ ID NO: 389 - RNA, 167 nt, Artificial Sequence
  Example 1.9
cuucacugauaaaguggagaaccgcuucaccaaaagcugucccuuaggggauuagaacuugagugaaggugggcugcuugcaucagccuaaugucgagaagugcuuucuucggaaaguaacccucgaaacaaagaaaggaaugcaaccacacacacagugggcuacc

SEQ ID NO: 390 - RNA, 140 nt, Artificial Sequence
  Example 1.10
accgcuucaccaauuaguugagugaaggugggcugcuugcaucagccuaaugucgagaagugcuuucuucggaaaguaacccucgaaacaaauucauuugaaagaaugaaggaaugcaaccacacacacagugggcuacc

SEQ ID NO: 391 - RNA, 147 nt, Artificial Sequence
  Example 1.11
accgcuucaccaaaagcugucccuuaggggauuagaacuugagugaaggugggcugcuugcaucagccuaaugucgagaagugcuuucuucggaaaguaacccucgaaacaaagaaaggaaugcaaccacacacacagugggcuacc

SEQ ID NO: 392 - RNA, 146 nt, Artificial Sequence
  Example 1.12
cuucacugauaaaguggagaaccgcuucaccaauuaguugagugaaggugggcugcuugcaucagccuaaugucgagaagugcuuucuucggaaaguaacccucgaaacaaagaaaggaaugcaaccacacacacagugggcuacc

SEQ ID NO: 393 - RNA, 126 nt, Artificial Sequence
  Example 1.13
accgcuucaccaauuaguugagugaaggugggcugcuugcaucagccuaaugucgagaagugcuuucuucggaaaguaacccucgaaacaaagaaaggaaugcaaccacacacacagugggcuacc

SEQ ID NO: 394 - RNA, 181 nt, Artificial Sequence
  Comparative Example 2.1
cuucacugauaaaguggagaaccgcuucaccaaaagcugucccuuaggggauuagaacuugagugaaggugggcugcuugcaucagccuaaugucgagaagugcuuucuucggaaaguaacccucgaaacaaauucauuugaaagaaugaaggaaugcaaccauccccaggacacacacac

SEQ ID NO: 395 - RNA, 174 nt, Artificial Sequence
  Example 2.1
gauaaaguggagaaccgcuucaccaaaagcugucccuuaggggauuagaacuugagugaaggugggcugcuugcaucagccuaaugucgagaagugcuuucuucggaaaguaacccucgaaacaaauucauuugaaagaaugaaggaaugcaaccauccccaggacacacacac

SEQ ID NO: 396 - RNA, 167 nt, Artificial Sequence
  Example 2.2
uggagaaccgcuucaccaaaagcugucccuuaggggauuagaacuugagugaaggugggcugcuugcaucagccuaaugucgagaagugcuuucuucggaaaguaacccucgaaacaaauucauuugaaagaaugaaggaaugcaaccauccccaggacacacacac

SEQ ID NO: 397 - RNA, 161 nt, Artificial Sequence
  Example 2.3
accgcuucaccaaaagcugucccuuaggggauuagaacuugagugaaggugggcugcuugcaucagccuaaugucgagaagugcuuucuucggaaaguaacccucgaaacaaauucauuugaaagaaugaaggaaugcaaccauccccaggacacacacac

SEQ ID NO: 398 - RNA, 175 nt, Artificial Sequence
  Example 2.4
cuucacugauaaaguggagaaccgcuucaccaaaagcuguuuagauuagaacuugagugaaggugggcugcuugcaucagccuaaugucgagaagugcuuucuucggaaaguaacccucgaaacaaauucauuugaaagaaugaaggaaugcaaccauccccaggacacacacac

SEQ ID NO: 399 - RNA, 170 nt, Artificial Sequence
  Example 2.5
cuucacugauaaaguggagaaccgcuucaccaaaagcuuuagagaacuugagugaaggugggcugcuugcaucagccuaaugucgagaagugcuuucuucggaaaguaacccucgaaacaaauucauuugaaagaaugaaggaaugcaaccauccccaggacacacacac

SEQ ID NO: 400 - RNA, 160 nt, Artificial Sequence
  Example 2.6
cuucacugauaaaguggagaaccgcuucaccaauuaguugagugaaggugggcugcuugcaucagccuaaugucgagaagugcuuucuucggaaaguaacccucgaaacaaauucauuugaaagaaugaaggaaugcaaccauccccaggacacacacac

SEQ ID NO: 401 - RNA, 177 nt, Artificial Sequence
  Example 2.7
cuucacugauaaaguggagaaccgcuucaccaaaagcugucccuuaggggauuagaacuugagugaaggugggcugcuugcaucagccuaaugucgagaagugcuuucuucggaaaguaacccucgaaacaaauucaugaaaaugaaggaaugcaaccauccccaggacacacacac

SEQ ID NO: 402 - RNA, 173 nt, Artificial Sequence
  Example 2.8
cuucacugauaaaguggagaaccgcuucaccaaaagcugucccuuaggggauuagaacuugagugaaggugggcugcuugcaucagccuaaugucgagaagugcuuucuucggaaaguaacccucgaaacaaauucgaaagaaggaaugcaaccauccccaggacacacacac

SEQ ID NO: 403 - RNA, 167 nt, Artificial Sequence
  Example 2.9
cuucacugauaaaguggagaaccgcuucaccaaaagcugucccuuaggggauuagaacuugagugaaggugggcugcuugcaucagccuaaugucgagaagugcuuucuucggaaaguaacccucgaaacaaagaaaggaaugcaaccauccccaggacacacacac

SEQ ID NO: 404 - RNA, 140 nt, Artificial Sequence
  Example 2.10
accgcuucaccaauuaguugagugaaggugggcugcuugcaucagccuaaugucgagaagugcuuucuucggaaaguaacccucgaaacaaauucauuugaaagaaugaaggaaugcaaccauccccaggacacacacac

SEQ ID NO: 405 - RNA, 147 nt, Artificial Sequence
  Example 2.11
accgcuucaccaaaagcugucccuuaggggauuagaacuugagugaaggugggcugcuugcaucagccuaaugucgagaagugcuuucuucggaaaguaacccucgaaacaaagaaaggaaugcaaccauccccaggacacacacac

SEQ ID NO: 406 - RNA, 146 nt, Artificial Sequence
  Example 2.12
cuucacugauaaaguggagaaccgcuucaccaauuaguugagugaaggugggcugcuugcaucagccuaaugucgagaagugcuuucuucggaaaguaacccucgaaacaaagaaaggaaugcaaccauccccaggacacacacac

SEQ ID NO: 407 - RNA, 126 nt, Artificial Sequence
  Example 2.13
accgcuucaccaauuaguugagugaaggugggcugcuugcaucagccuaaugucgagaagugcuuucuucggaaaguaacccucgaaacaaagaaaggaaugcaaccauccccaggacacacacac

SEQ ID NO: 408 - RNA, 181 nt, Artificial Sequence
  Comparative Example 3.1
cuucacugauaaaguggagaaccgcuucaccaaaagcugucccuuaggggauuagaacuugagugaaggugggcugcuugcaucagccuaaugucgagaagugcuuucuucggaaaguaacccucgaaacaaauucauuugaaagaaugaaggaaugcaacagaacacauaccccugggcc

SEQ ID NO: 409 - RNA, 174 nt, Artificial Sequence
  Example 3.1
gauaaaguggagaaccgcuucaccaaaagcugucccuuaggggauuagaacuugagugaaggugggcugcuugcaucagccuaaugucgagaagugcuuucuucggaaaguaacccucgaaacaaauucauuugaaagaaugaaggaaugcaacagaacacauaccccugggcc

SEQ ID NO: 410 - RNA, 167 nt, Artificial Sequence
  Example 3.2
uggagaaccgcuucaccaaaagcugucccuuaggggauuagaacuugagugaaggugggcugcuugcaucagccuaaugucgagaagugcuuucuucggaaaguaacccucgaaacaaauucauuugaaagaaugaaggaaugcaacagaacacauaccccugggcc

SEQ ID NO: 411 - RNA, 161 nt, Artificial Sequence
  Example 3.3
accgcuucaccaaaagcugucccuuaggggauuagaacuugagugaaggugggcugcuugcaucagccuaaugucgagaagugcuuucuucggaaaguaacccucgaaacaaauucauuugaaagaaugaaggaaugcaacagaacacauaccccugggcc

SEQ ID NO: 412 - RNA, 175 nt, Artificial Sequence
  Example 3.4
cuucacugauaaaguggagaaccgcuucaccaaaagcuguuuagauuagaacuugagugaaggugggcugcuugcaucagccuaaugucgagaagugcuuucuucggaaaguaacccucgaaacaaauucauuugaaagaaugaaggaaugcaacagaacacauaccccugggcc

SEQ ID NO: 413 - RNA, 170 nt, Artificial Sequence
  Example 3.5
cuucacugauaaaguggagaaccgcuucaccaaaagcuuuagagaacuugagugaaggugggcugcuugcaucagccuaaugucgagaagugcuuucuucggaaaguaacccucgaaacaaauucauuugaaagaaugaaggaaugcaacagaacacauaccccugggcc

SEQ ID NO: 414 - RNA, 160 nt, Artificial Sequence
  Example 3.6
cuucacugauaaaguggagaaccgcuucaccaauuaguugagugaaggugggcugcuugcaucagccuaaugucgagaagugcuuucuucggaaaguaacccucgaaacaaauucauuugaaagaaugaaggaaugcaacagaacacauaccccugggcc

SEQ ID NO: 415 - RNA, 177 nt, Artificial Sequence
  Example 3.7
cuucacugauaaaguggagaaccgcuucaccaaaagcugucccuuaggggauuagaacuugagugaaggugggcugcuugcaucagccuaaugucgagaagugcuuucuucggaaaguaacccucgaaacaaauucaugaaaaugaaggaaugcaacagaacacauaccccugggcc

SEQ ID NO: 416 - RNA, 173 nt, Artificial Sequence
  Example 3.8
cuucacugauaaaguggagaaccgcuucaccaaaagcugucccuuaggggauuagaacuugagugaaggugggcugcuugcaucagccuaaugucgagaagugcuuucuucggaaaguaacccucgaaacaaauucgaaagaaggaaugcaacagaacacauaccccugggcc

SEQ ID NO: 417 - RNA, 167 nt, Artificial Sequence
  Example 3.9
cuucacugauaaaguggagaaccgcuucaccaaaagcugucccuuaggggauuagaacuugagugaaggugggcugcuugcaucagccuaaugucgagaagugcuuucuucggaaaguaacccucgaaacaaagaaaggaaugcaacagaacacauaccccugggcc

SEQ ID NO: 418 - RNA, 140 nt, Artificial Sequence
  Example 3.10
accgcuucaccaauuaguugagugaaggugggcugcuugcaucagccuaaugucgagaagugcuuucuucggaaaguaacccucgaaacaaauucauuugaaagaaugaaggaaugcaacagaacacauaccccugggcc

SEQ ID NO: 419 - RNA, 147 nt, Artificial Sequence
  Example 3.11
accgcuucaccaaaagcugucccuuaggggauuagaacuugagugaaggugggcugcuugcaucagccuaaugucgagaagugcuuucuucggaaaguaacccucgaaacaaagaaaggaaugcaacagaacacauaccccugggcc

SEQ ID NO: 420 - RNA, 146 nt, Artificial Sequence
  Example 3.12
cuucacugauaaaguggagaaccgcuucaccaauuaguugagugaaggugggcugcuugcaucagccuaaugucgagaagugcuuucuucggaaaguaacccucgaaacaaagaaaggaaugcaacagaacacauaccccugggcc

SEQ ID NO: 421 - RNA, 126 nt, Artificial Sequence
  Example 3.13
accgcuucaccaauuaguugagugaaggugggcugcuugcaucagccuaaugucgagaagugcuuucuucggaaaguaacccucgaaacaaagaaaggaaugcaacagaacacauaccccugggcc

SEQ ID NO: 422 - DNA, 20 bp, Artificial Sequence
  protospacer sequence for targeting DY2
cacacacacagtgggctacc

SEQ ID NO: 423 - DNA, 20 bp, Artificial Sequence
  protospacer sequence for targeting DY10
catccccaggacacacacac

SEQ ID NO: 424 - DNA, 20 bp, Artificial Sequence
  protospacer sequence for targeting Intergenic-22
agaacacatacccctgggcc

SEQ ID NO: 425 - RNA, 10 nt, Artificial Sequence
  Linker variation, MF
uucgaaagaa

SEQ ID NO: 426 - RNA, 12 nt, Artificial Sequence
  Linker variation, MF
uucagaaaugaa

SEQ ID NO: 427 - RNA, 14 nt, Artificial Sequence
  Linker variation, MF
uucaugaaaaugaa

SEQ ID NO: 428 - RNA, 16 nt, Artificial Sequence
  Linker variation, MF
uucauugaaaaaugaa

SEQ ID NO: 429 - RNA, 18 nt, Artificial Sequence
  Linker variation, MF
uucauuugaaagaaugaa

SEQ ID NO: 430 - RNA, 24 nt, Artificial Sequence
  Second region, 13bp deletion
ccgcuucacuuagagugaaggugg

SEQ ID NO: 431 - RNA, 26 nt, Artificial Sequence
  Second region, 12bp deletion
ccgcuucaccuuaggagugaaggugg

SEQ ID NO: 432 - RNA, 9 nt, Artificial Sequence
  second region, 5' remains
ccgcuucac

SEQ ID NO: 433 - RNA, 11 nt, Artificial Sequence
  second region, 3' remains
agugaaggugg

SEQ ID NO: 434 - RNA, 29 nt, Artificial Sequence
  intermediate sequence of the second region
aaaagcugucccuuaggggauuagaacuu

SEQ ID NO: 435 - RNA, 31 nt, Artificial Sequence
  intermediate sequence of the second region
caaaagcugucccuuaggggauuagaacuug

SEQ ID NO: 436 - RNA, 120 nt, Artificial Sequence
  Example 1.14
accgcuucacuuagagugaaggugggcugcuugcaucagccuaaugucgagaagugcuuucuucggaaaguaacccucgaaacaaagaaaggaaugcaaccacacacacagugggcuacc

SEQ ID NO: 437 - RNA, 120 nt, Artificial Sequence
  Example 2.14
accgcuucacuuagagugaaggugggcugcuugcaucagccuaaugucgagaagugcuuucuucggaaaguaacccucgaaacaaagaaaggaaugcaaccauccccaggacacacacac

SEQ ID NO: 438 - RNA, 120 nt, Artificial Sequence
  Example 3.14
accgcuucacuuagagugaaggugggcugcuugcaucagccuaaugucgagaagugcuuucuucggaaaguaacccucgaaacaaagaaaggaaugcaacagaacacauaccccugggcc

SEQ ID NO: 439 - RNA, 120 nt, Artificial Sequence
  engineered sgRNA
accgcuucacuuagagugaaggugggcugcuugcaucagccuaaugucgagaagugcuuucuucggaaaguaacccucgaaacaaagaaaggaaugcaacnnnnnnnnnnnnnnnnnnnn

SEQ ID NO: 440 - RNA, 12 nt, Artificial Sequence
  Upper deleted part of second region
aaaagcuguccc

SEQ ID NO: 441 - RNA, 13 nt, Artificial Sequence
  Lower deleted part of second region
caaaagcuguccc